European Patent Application EP 4 266 058 A2, published October 25, 2023. Title: GENETICALLY ENCODED SYSTEM FOR CONSTRUCTING AND DETECTING BIOLOGICALLY ACTIVE AGENTS. Applicant: The Regents Of The University Of Colorado. Application EP 19831095.5. The sequence listing filed with the application follows.

SEQUENCE LISTING (104 sequences)

SEQ ID NO: 1 - protein, 27 aa, synthetic construct
  REGION 1..27: note = Synthetic Polypeptide
MGDSSVQDQWKELSHEDLEPPPEHIPP

SEQ ID NO: 2 - protein, 27 aa, synthetic construct
  REGION 1..27: note = Synthetic Polypeptide
ESFDDELRRKEMRRGIDLATTLERIEK

SEQ ID NO: 3 - protein, 298 aa, synthetic construct
  REGION 1..298: note = Synthetic Polypeptide
MEMEKEFEQIDKSGSWAAIYQDIRHEASDFPCRVAKLPKNKNRNRYRDVSPFDHSRIKLHQEDNDYINASLIKMEEAQRSYILTQGPLPNTCGHFWEMVWEQKSRGVVMLNRVMEKGSLKCAQYWPQKEEKEMIFEDTNLKLTLISEDIKSYYTVRQLELENLTTQETREILHFHYTTWPDFGVPESPASFLNFLFKVRESGSLSPEHGPVVVHCSAGIGRSGTFCLADTCLLLMDKRKDPSSVDIKKVLLEMRKFRMGLIQTADQLRFSYLAVIEGAKFIMGDSSVQDQWKELSHED

SEQ ID NO: 4 - protein, 303 aa, synthetic construct
  REGION 1..303: note = Synthetic Polypeptide
LELNKKQESEDTAKAGFWEEFESLQKQEVKNLHQRLEGQRPENKGKNRYKNILPFDHSRVILQGRDSNIPGSDYINANYIKNQLLGPDENAKTYIASQGCLEATVNDFWQMAWQENSRVIVMTTREVEKGRNKCVPYWPEVGMQRAYGPYSVTNCGEHDTTEYKLRTLQVSPLDNGDLIREIWHYQYLSWPDHGVPSEPGGVLSFLDQINQRQESLPHAGPIIVHCSAGIGRTGTIIVIDMLMENISTKGLDCDIDIQKTIQMVRAQRSGMVQTEAQYKFIYVAIAQFIETTKKKLEVLQSQK

SEQ ID NO: 5 - protein, 10 aa, synthetic construct
  REGION 1..10: note = Synthetic Polypeptide
LSHEDLATTL

SEQ ID NO: 6 - protein, 5 aa, synthetic construct
  REGION 1..5: note = Synthetic Polypeptide
LSHED

SEQ ID NO: 7 - protein, 5 aa, synthetic construct
  REGION 1..5: note = Synthetic Polypeptide
LATTL

SEQ ID NO: 8 - protein, 9 aa, synthetic construct
  REGION 1..9: note = Synthetic Polypeptide
LSHEDATTL

SEQ ID NO: 9 - protein, 8 aa, synthetic construct
  REGION 1..8: note = Synthetic Polypeptide
LSHEDTTL

SEQ ID NO: 10 - protein, 13 aa, synthetic construct
  REGION 1..13: note = Synthetic Polypeptide
  MOD_RES 7: note = phosphorylated
ETGTEEYMKMDLG

SEQ ID NO: 11 - protein, 13 aa, synthetic construct
  REGION 1..13: note = Synthetic Polypeptide
  MOD_RES 9: note = phosphorylated
RRLIEDAEYAARG

SEQ ID NO: 12 - DNA, 1347 bp, synthetic construct
  misc_feature 1..1347: note = Synthetic Polynucleotide
  source 1..1347: mol_type = other DNA
atggagatggaaaaggagttcgagcagatcgacaagtccgggagctgggcggccatttaccaggatatccgacatgaagccagtgacttcccatgtagagtggccaagcttcctaagaacaaaaaccgaaataggtacagagacgtcagtccctttgaccatagtcggattaaactacatcaagaagataatgactatatcaacgctagtttgataaaaatggaagaagcccaaaggagttacattcttacccagggccctttgcctaacacatgcggtcacttttgggagatggtgtgggagcagaaaagcaggggtgtcgtcatgctcaacagagtgatggagaaaggttcgttaaaatgcgcacaatactggccacaaaaagaagaaaaagagatgatctttgaagacacaaatttgaaattaacattgatctctgaagatatcaagtcatattatacagtgcgacagctagaattggaaaaccttacaacccaagaaactcgagagatcttacatttccactataccacatggcctgactttggagtccctgaatcaccagcctcattcttgaactttcttttcaaagtccgagagtcagggtcactcagcccggagcacgggcccgttgtggtgcactgcagtgcaggcatcggcaggtctggaaccttctgtctggctgatacctgcctcttgctgatggacaagaggaaagacccttcttccgttgatatcaagaaagtgctgttagaaatgaggaagtttcggatggggctgatccagacagccgaccagctgcgcttctcctacctggctgtgatcgaaggtgccaaattcatcatgggggactcttccgtgcaggatcagtggaaggagctttcccacgaggacgctgctacacttgaacgtattgagaagaactttgtcattactgacccaaggttgccagataatcccattatattcgcgtccgatagtttcttgcagttgacagaatatagccgtgaagaaattttgggaagaaactgcaggtttctacaaggtcctgaaactgatcgcgcgacagtgagaaaaattagagatgccatagataaccaaacagaggtcactgttcagctgattaattatacaaagagtggtaaaaagttctggaacctctttcacttgcagcctatgcgagatcagaagggagatgtccagtactttattggggttcagttggatggaactgagcatgtccgagatgctgccgagagagagggagtcatgctgattaagaaaactgcagaaaatattgatgaggcggcaaaagaacttctcgagcaccaccaccaccaccactga

SEQ ID NO: 13 - protein, 448 aa, synthetic construct
  REGION 1..448: note = Synthetic Polypeptide
MEMEKEFEQIDKSGSWAAIYQDIRHEASDFPCRVAKLPKNKNRNRYRDVSPFDHSRIKLHQEDNDYINASLIKMEEAQRSYILTQGPLPNTCGHFWEMVWEQKSRGVVMLNRVMEKGSLKCAQYWPQKEEKEMIFEDTNLKLTLISEDIKSYYTVRQLELENLTTQETREILHFHYTTWPDFGVPESPASFLNFLFKVRESGSLSPEHGPVVVHCSAGIGRSGTFCLADTCLLLMDKRKDPSSVDIKKVLLEMRKFRMGLIQTADQLRFSYLAVIEGAKFIMGDSSVQDQWKELSHEDAATLERIEKNFVITDPRLPDNPIIFASDSFLQLTEYSREEILGRNCRFLQGPETDRATVRKIRDAIDNQTEVTVQLINYTKSGKKFWNLFHLQPMRDQKGDVQYFIGVQLDGTEHVRDAAEREGVMLIKKTAENIDEAAKELLEHHHHHH

SEQ ID NO: 14 - DNA, 1347 bp, synthetic construct
  misc_feature 1..1347: note = Synthetic Polynucleotide
  source 1..1347: mol_type = other DNA
atggagatggaaaaggagttcgagcagatcgacaagtccgggagctgggcggccatttaccaggatatccgacatgaagccagtgacttcccatgtagagtggccaagcttcctaagaacaaaaaccgaaataggtacagagacgtcagtccctttgaccatagtcggattaaactacatcaagaagataatgactatatcaacgctagtttgataaaaatggaagaagcccaaaggagttacattcttacccagggccctttgcctaacacatgcggtcacttttgggagatggtgtgggagcagaaaagcaggggtgtcgtcatgctcaacagagtgatggagaaaggttcgttaaaatgcgcacaatactggccacaaaaagaagaaaaagagatgatctttgaagacacaaatttgaaattaacattgatctctgaagatatcaagtcatattatacagtgcgacagctagaattggaaaaccttacaacccaagaaactcgagagatcttacatttccactataccacatggcctgactttggagtccctgaatcaccagcctcattcttgaactttcttttcaaagtccgagagtcagggtcactcagcccggagcacgggcccgttgtggtgcactgcagtgcaggcatcggcaggtctggaaccttctgtctggctgatacctgcctcttgctgatggacaagaggaaagacccttcttccgttgatatcaagaaagtgctgttagaaatgaggaagtttcggatggggctgatccagacagccgaccagctgcgcttctcctacctggctgtgatcgaaggtgccaaattcatcatgggggactctgccgtgcaggatcagtggaaggagctttcccacgaggacgctactacacttgaacgtattgagaagaactttgtcattactgacccaaggttgccagataatcccattatattcgcgtccgatagtttcttgcagttgacagaatatagccgtgaagaaattttgggaagaaactgcaggtttctacaaggtcctgaaactgatcgcgcgacagtgagaaaaattagagatgccatagataaccaaacagaggtcactgttcagctgattaattatacaaagagtggtaaaaagttctggaacctctttcacttgcagcctatgcgagatcagaagggagatgtccagtactttattggggttcagttggatggaactgagcatgtccgagatgctgccgagagagagggagtcatgctgattaagaaaactgcagaaaatattgatgaggcggcaaaagaacttctcgagcaccaccaccaccaccactga

SEQ ID NO: 15 - protein, 448 aa, synthetic construct
  REGION 1..448: note = Synthetic Polypeptide
MEMEKEFEQIDKSGSWAAIYQDIRHEASDFPCRVAKLPKNKNRNRYRDVSPFDHSRIKLHQEDNDYINASLIKMEEAQRSYILTQGPLPNTCGHFWEMVWEQKSRGVVMLNRVMEKGSLKCAQYWPQKEEKEMIFEDTNLKLTLISEDIKSYYTVRQLELENLTTQETREILHFHYTTWPDFGVPESPASFLNFLFKVRESGSLSPEHGPVVVHCSAGIGRSGTFCLADTCLLLMDKRKDPSSVDIKKVLLEMRKFRMGLIQTADQLRFSYLAVIEGAKFIMGDSAVQDQWKELSHEDATTLERIEKNFVITDPRLPDNPIIFASDSFLQLTEYSREEILGRNCRFLQGPETDRATVRKIRDAIDNQTEVTVQLINYTKSGKKFWNLFHLQPMRDQKGDVQYFIGVQLDGTEHVRDAAEREGVMLIKKTAENIDEAAKELLEHHHHHH

SEQ ID NO: 16 - DNA, 1350 bp, synthetic construct
  misc_feature 1..1350: note = Synthetic Polynucleotide
  source 1..1350: mol_type = other DNA
atgcccaccaccatcgagcgggagttcgaagagttggatactcagcgtcgctggcagccgctgtacttggaaattcgaaatgagtcccatgactatcctcatagagtggccaagtttccagaaaacagaaatcgaaacagatacagagatgtaagcccatatgatcacagtcgtgttaaactgcaaaatgctgagaatgattatattaatgccagtttagttgacatagaagaggcacaaaggagttacatcttaacacagggtccacttcctaacacatgctgccatttctggcttatggtttggcagcagaagaccaaagcagttgtcatgctgaaccgcgtgatggagaaaggttcgttaaaatgtgcacagtactggccaacagatgaccaagagatgctgtttaaagaaacaggattcagtgtgaagctcttgtcagaagatgtgaagtcgtattatacagtacatctactacaattagaaaatatcaatagtggtgaaaccagaacaatatctcactttcattatactacctggccagattttggagtccctgaatcaccagcttcatttctcaatttcttgtttaaagtgagagaatctggctccttgaaccctgaccatgggcctgcggtgatccactgtagtgcaggcattgggcgctctggcaccttctctctggtagacacttgtcttttgctgatggacaagaggaaagacccttcttccgttgatatcaagaaagtgctgttagaaatgaggaagtttcggatggggctgatccagacagccgaccagctgcgcttctcctacctggctgtgatcgaaggtgccaaattcatcatgggggactcttccgtgcaggatcagtggaaggagctttcccacgaggacgctgctacacttgaacgtattgagaagaactttgtcattactgacccaaggttgccagataatcccattatattcgcgtccgatagtttcttgcagttgacagaatatagccgtgaagaaattttgggaagaaactgcaggtttctacaaggtcctgaaactgatcgcgcgacagtgagaaaaattagagatgccatagataaccaaacagaggtcactgttcagctgattaattatacaaagagtggtaaaaagttctggaacctctttcacttgcagcctatgcgagatcagaagggagatgtccagtactttattggggttcagttggatggaactgagcatgtccgagatgctgccgagagagagggagtcatgctgattaagaaaactgcagaaaatattgatgaggcggcaaaagaacttctcgagcaccaccaccaccaccactga

SEQ ID NO: 17 - protein, 449 aa, synthetic construct
  REGION 1..449: note = Synthetic Polypeptide
MPTTIEREFEELDTQRRWQPLYLEIRNESHDYPHRVAKFPENRNRNRYRDVSPYDHSRVKLQNAENDYINASLVDIEEAQRSYILTQGPLPNTCCHFWLMVWQQKTKAVVMLNRVMEKGSLKCAQYWPTDDQEMLFKETGFSVKLLSEDVKSYYTVHLLQLENINSGETRTISHFHYTTWPDFGVPESPASFLNFLFKVRESGSLNPDHGPAVIHCSAGIGRSGTFSLVDTCLLLMDKRKDPSSVDIKKVLLEMRKFRMGLIQTADQLRFSYLAVIEGAKFIMGDSSVQDQWKELSHEDAATLERIEKNFVITDPRLPDNPIIFASDSFLQLTEYSREEILGRNCRFLQGPETDRATVRKIRDAIDNQTEVTVQLINYTKSGKKFWNLFHLQPMRDQKGDVQYFIGVQLDGTEHVRDAAEREGVMLIKKTAENIDEAAKELLEHHHHHH

SEQ ID NO: 18 - DNA, 1350 bp, synthetic construct
  misc_feature 1..1350: note = Synthetic Polynucleotide
  source 1..1350: mol_type = other DNA
atgcccaccaccatcgagcgggagttcgaagagttggatactcagcgtcgctggcagccgctgtacttggaaattcgaaatgagtcccatgactatcctcatagagtggccaagtttccagaaaacagaaatcgaaacagatacagagatgtaagcccatatgatcacagtcgtgttaaactgcaaaatgctgagaatgattatattaatgccagtttagttgacatagaagaggcacaaaggagttacatcttaacacagggtccacttcctaacacatgctgccatttctggcttatggtttggcagcagaagaccaaagcagttgtcatgctgaaccgcattgtggagaaagaatcggttaaatgtgcacagtactggccaacagatgaccaagagatgctgtttaaagaaacaggattcagtgtgaagctcttgtcagaagatgtgaagtcgtattatacagtacatctactacaattagaaaatatcaatagtggtgaaaccagaacaatatctcactttcattatactacctggccagattttggagtccctgaatcaccagcttcatttctcaatttcttgtttaaagtgagagaatctggctccttgaaccctgaccatgggcctgcggtgatccactgtagtgcaggcattgggcgctctggcaccttctctctggtagacacttgtcttttgctgatggacaagaggaaagacccttcttccgttgatatcaagaaagtgctgttagaaatgaggaagtttcggatggggctgatccagacagccgaccagctgcgcttctcctacctggctgtgatcgaaggtgccaaattcatcatgggggactcttccgtgcaggatcagtggaaggagctttcccacgaggacgctgctacacttgaacgtattgagaagaactttgtcattactgacccaaggttgccagataatcccattatattcgcgtccgatagtttcttgcagttgacagaatatagccgtgaagaaattttgggaagaaactgcaggtttctacaaggtcctgaaactgatcgcgcgacagtgagaaaaattagagatgccatagataaccaaacagaggtcactgttcagctgattaattatacaaagagtggtaaaaagttctggaacctctttcacttgcagcctatgcgagatcagaagggagatgtccagtactttattggggttcagttggatggaactgagcatgtccgagatgctgccgagagagagggagtcatgctgattaagaaaactgcagaaaatattgatgaggcggcaaaagaacttctcgagcaccaccaccaccaccactga

SEQ ID NO: 19 - protein, 449 aa, synthetic construct
  REGION 1..449: note = Synthetic Polypeptide
MPTTIEREFEELDTQRRWQPLYLEIRNESHDYPHRVAKFPENRNRNRYRDVSPYDHSRVKLQNAENDYINASLVDIEEAQRSYILTQGPLPNTCCHFWLMVWQQKTKAVVMLNRIVEKESVKCAQYWPTDDQEMLFKETGFSVKLLSEDVKSYYTVHLLQLENINSGETRTISHFHYTTWPDFGVPESPASFLNFLFKVRESGSLNPDHGPAVIHCSAGIGRSGTFSLVDTCLLLMDKRKDPSSVDIKKVLLEMRKFRMGLIQTADQLRFSYLAVIEGAKFIMGDSSVQDQWKELSHEDAATLERIEKNFVITDPRLPDNPIIFASDSFLQLTEYSREEILGRNCRFLQGPETDRATVRKIRDAIDNQTEVTVQLINYTKSGKKFWNLFHLQPMRDQKGDVQYFIGVQLDGTEHVRDAAEREGVMLIKKTAENIDEAAKELLEHHHHHH

SEQ ID NO: 20 - DNA, 1827 bp, synthetic construct
  misc_feature 1..1827: note = Synthetic Polynucleotide
  source 1..1827: mol_type = other DNA
atgcatcatcatcatcatcatgtgagcaagggcgaggagctgttcaccggggtggtgcccatcctggtcgagctggacggcgacgtaaacggccacaagttcagcgtccgcggcgagggcgagggcgatgccaccaacggcaagctgaccctgaagttcatctgcaccaccggcaagctgcccgtgccctggcccaccctcgtgaccaccttcggctacggcgtggcctgcttcagccgctaccccgaccacatgaagcagcacgacttcttcaagtccgccatgcccgaaggctacgtccaggagcgcaccatctctttcaaggacgacggtacctacaagacccgcgccgaggtgaagttcgagggcgacaccctggtgaaccgcatcgagctgaagggcatcgacttcaaggaggacggcaacatcctggggcacaagctggagtacaacttcaacagccactacgtctatatcacggccgacaagcagaagaactgcatcaaggctaacttcaagatccgccacaacgttgaggacggcagcgtgcagctcgccgaccactaccagcagaacacccccatcggcgacggccccgtgctgctgcccgacaaccactacctgagccatcagtccaagctgagcaaagaccccaacgagaagcgcgatcacatggtcctgctggagttcgtgaccgccgccgggattacacatggcatggacgagctgtacaagtggtattttgggaagatcactcgtcgggagtccgagcggctgctgctcaaccccgaaaacccccggggaaccttcttggtccgggagagcgagacgacaaaaggtgcctattgcctctccgtttctgactttgacaacgccaaggggctcaatgtgaagcactacaagatccgcaagctggacagcggcggcttctacatcacctcacgcacacagttcagcagcctgcagcagctggtggcctactactccaaacatgctgatggcttgtgccaccgcctgactaacgtctgtgggtctacatctggatctgggaagccgggttctggtgagggttcttggatggaggactatgactacgtccacctacagggggagctcgtgtctaagggcgaagagctgatcaaggaaaatatgcgtatgaaggtggtcatggaaggttcggtcaacggccaccaattcaaatgcacaggtgaaggagaaggcagaccgtacgagggaactcaaaccatgaggatcaaagtcatcgagggaggacccctgccatttgcctttgacattcttgccacgtcgttcatgtatggcagccgtacttttatcaagtacccggccgacatccctgatttctttaaacagtcctttcctgagggttttacttgggaaagagttacgagatacgaagatggtggagtcgtcaccgtcacgcaggacaccagccttgaggatggcgagctcgtctacaacgtcaaggtcagaggggtaaactttccctccaatggtcccgtgatgcagaagaagaccaagggttgggagcctaatacagagatgatgtatccagcagatggtggtctgagaggatacactgacatcgcactgaaagttgatggtggtggccatctgcactgcaacttcgtgacaacttacaggtcaaaaaagaccgtcgggaacatcaagatgcccggtgtccatgccgttgatcaccgcctggaaaggatcgaggagagtgacaatgaaacctacgtagtgcaacgcgaagtggcagttgccaaatacagcaaccttggtggtggcatggacgagctgtacaagtaa

SEQ ID NO: 21 - protein, 608 aa, synthetic construct
  REGION 1..608: note = Synthetic Polypeptide
MHHHHHHVSKGEELFTGVVPILVELDGDVNGHKFSVRGEGEGDATNGKLTLKFICTTGKLPVPWPTLVTTFGYGVACFSRYPDHMKQHDFFKSAMPEGYVQERTISFKDDGTYKTRAEVKFEGDTLVNRIELKGIDFKEDGNILGHKLEYNFNSHYVYITADKQKNCIKANFKIRHNVEDGSVQLADHYQQNTPIGDGPVLLPDNHYLSHQSKLSKDPNEKRDHMVLLEFVTAAGITHGMDELYKWYFGKITRRESERLLLNPENPRGTFLVRESETTKGAYCLSVSDFDNAKGLNVKHYKIRKLDSGGFYITSRTQFSSLQQLVAYYSKHADGLCHRLTNVCGSTSGSGKPGSGEGSWMEDYDYVHLQGELVSKGEELIKENMRMKVVMEGSVNGHQFKCTGEGEGRPYEGTQTMRIKVIEGGPLPFAFDILATSFMYGSRTFIKYPADIPDFFKQSFPEGFTWERVTRYEDGGVVTVTQDTSLEDGELVYNVKVRGVNFPSNGPVMQKKTKGWEPNTEMMYPADGGLRGYTDIALKVDGGGHLHCNFVTTYRSKKTVGNIKMPGVHAVDHRLERIEESDNETYVVQREVAVAKYSNLGGGMDELYK

SEQ ID NO: 22 - DNA, 70 bp, synthetic construct
  misc_feature 1..70: note = Synthetic Polynucleotide
  source 1..70: mol_type = other DNA
gcaaatgggcggtaggcgtgtacggtgggaggtctatataagcagagctggtttagtgaaccgtcagatc

SEQ ID NO: 23 - DNA, 66 bp, synthetic construct
  misc_feature 1..66: note = Synthetic Polynucleotide
  source 1..66: mol_type = other DNA
ggcagcggcgccaccaacttctccctgctgaagcaggccggcgacgtggaggagaaccccggcccc

SEQ ID NO: 24 - protein, 22 aa, synthetic construct
  REGION 1..22: note = Synthetic Polypeptide
GSGATNFSLLKQAGDVEENPGP

SEQ ID NO: 25 - DNA, 160 bp, synthetic construct
  misc_feature 1..160: note = Synthetic Polynucleotide
  source 1..160: mol_type = other DNA
ttctagagcacagctaacaccacgtcgtccctatctgctgccctaggtctatgagtggttgctggataactttacgggcatgcataaggctcggtatctatattcagggagaccacaacggtttccctctacaaataattttgtttaacttttactagag

SEQ ID NO: 26 - DNA, 153 bp, synthetic construct
  misc_feature 1..153: note = Synthetic Polynucleotide
  source 1..153: mol_type = other DNA
gcacagctaacaccacgtcgtccctatctgctgccctaggtctatgagtggttgctggataactttacgggcatgcataaggctcgtataatatattcagggagaccacaacggtttccctctacaaataattttgtttaacttttactagag

SEQ ID NO: 27 - DNA, 304 bp, synthetic construct
  misc_feature 1..304: note = Synthetic Polynucleotide
  source 1..304: mol_type = other DNA
agaaaccaattgtccatattgcatcagacattgccgtcactgcgtcttttactggctcttctcgctaaccaaaccggtaaccccgcttattaaaagcattctgtaacaaagcgggaccaaagccatgacaaaaacgcgtaacaaaagtgtctataatcacggcagaaaagtccacattgattatttgcacggcgtcacactttgctatgccatagcatttttatccataagattagcggatcctacctgacgctttttatcgcaactctctactgtttctccatacccgtttttttgggctagc

SEQ ID NO: 28 - DNA, 72 bp, synthetic construct
  misc_feature 1..72: note = Synthetic Polynucleotide
  source 1..72: mol_type = other DNA
acaagaaagtttgttcattaggcaccccgggctttactcgtaaagcttccggcgcgtatgttgtgtcgaccg

SEQ ID NO: 29 - DNA, 246 bp, synthetic construct
  misc_feature 1..246: note = Synthetic Polynucleotide
  source 1..246: mol_type = other DNA
cgactgcacggtgcaccaatgcttctggcgtcaggcagccatcggaagctgtggtatggctgtgcaggtcgtaaatcactgcataattcgtgtcgctcaaggcgcactcccgttctggataatgttttttgcgccgacatcataacggttctggcaaatattctgaaatgagctgttgacaattaatcatccggctcgtataatgtgtggaattgtgagcggataacaatttcacacaggaaacag

SEQ ID NO: 30 - DNA, 19 bp, synthetic construct
  misc_feature 1..19: note = Synthetic Polynucleotide
  source 1..19: mol_type = other DNA
cctatagtgagtcgtatta

SEQ ID NO: 31 - DNA, 18 bp, synthetic construct
  misc_feature 1..18: note = Synthetic Polynucleotide
  source 1..18: mol_type = other DNA
ttaaagaggagaaaggtc

SEQ ID NO: 32 - DNA, 24 bp, synthetic construct
  misc_feature 1..24: note = Synthetic Polynucleotide
  source 1..24: mol_type = other DNA
cgaaaaaaagtaaggcggtaatcc

SEQ ID NO: 33 - DNA, 23 bp, synthetic construct
  misc_feature 1..23: note = Synthetic Polynucleotide
  source 1..23: mol_type = other DNA
tgcagaaagaggagaaatactag

SEQ ID NO: 34 - DNA, 21 bp, synthetic construct
  misc_feature 1..21: note = Synthetic Polynucleotide
  source 1..21: mol_type = other DNA
attaaagaggagaaatactag

SEQ ID NO: 35 - DNA, 22 bp, synthetic construct
  misc_feature 1..22: note = Synthetic Polynucleotide
  source 1..22: mol_type = other DNA
gtgcagtaaggaggaaaaaaaa

SEQ ID NO: 36 - DNA, 25 bp, synthetic construct
  misc_feature 1..25: note = Synthetic Polynucleotide
  source 1..25: mol_type = other DNA
gctagctttaagaaggagatatacc

SEQ ID NO: 37 - protein, 94 aa, synthetic construct
  REGION 1..94: note = Synthetic Polypeptide
MARVTVQDAVEKIGNRFDLVLVAARRARQMQVGGKDPLVPEENDKTTVIALREIEEGLINNQILDVRERQEQQEQEAAELQAVTAIAEGRRAAA

SEQ ID NO: 38 - protein, 218 aa, synthetic construct
  REGION 1..218: note = Synthetic Polypeptide
MSISSRVKSKRIQLGLNQAELAQKVGTTQQSIEQLENGKTKRPRFLPELASALGVSVDWLLNGTSDSNVRFVGHVEPKGKYPLISMVRARSWCEACEPYDIKDIDEWYDSDVNLLGNGFWLKVEGDSMTSPVGQSIPEGHMVLVDTGREPVNGSLVVAKLTDANEATFKKLVIDGGQKYLKGLNPSWPMTPINGNCKIIGVVVEARVKFVDYKDDDDK

SEQ ID NO: 39 - protein, 98 aa, synthetic construct
  REGION 1..98: note = Synthetic Polypeptide
WYFGKITRRESERLLLNPENPRGTFLVRESETVKGAYALSVSDFDNAKGLNVKHYLIRKLDSGGFYITSRTQFSSLQQLVAYYSKHADGLCHRLTNVC

SEQ ID NO: 40 - protein, 12 aa, synthetic construct
  REGION 1..12: note = Synthetic Polypeptide
WMEDYDYVHLQG

SEQ ID NO: 41 - protein, 11 aa, synthetic construct
  REGION 1..11: note = Synthetic Polypeptide
EPQYEEIPIYL

SEQ ID NO: 42 - protein, 10 aa, synthetic construct
  REGION 1..10: note = Synthetic Polypeptide
DHQYYNDFPG

SEQ ID NO: 43 - protein, 10 aa, synthetic construct
  REGION 1..10: note = Synthetic Polypeptide
PQRYLVIQGD

SEQ ID NO: 44 - protein, 287 aa, synthetic construct
  REGION 1..287: note = Synthetic Polypeptide
MSKPQTQGLAKDAWEIPRESLRLEVKLGQGCFGEVWMGTWNGTTRVAIKTLKPGTMSPEAFLQEAQVMKKLRHEKLVQLYAVVSEEPIYIVTEYMSKGSLLDFLKGETGKYLRLPQLVDMAAQIASGMAYVERMNYVHRDLRAANILVGENLVCKVADFGLARLIEDNEYTARQGAKFPIKWTAPEAALYGRFTIKSDVWSFGILLTELTTKGRVPYPGMVNREVLDQVERGYRMPCPPECPESLHDLMCQCWRKEPEERPTFEYLQAFLEDYFTSTEPQYQPGENL

SEQ ID NO: 45 - protein, 378 aa, synthetic construct
  REGION 1..378: note = Synthetic Polypeptide
MVDYSVWDHIEVSDDEDETHPNIDTASLFRWRHQARVERMEQFQKEKEELDRGCRECKRKVAECQRKLKELEVAEGGKAELERLQAEAQQLRKEERSWEQKLEEMRKKEKSMPWNVDTLSKDGFSKSMVNTKPEKTEEDSEEVREQKHKTFVEKYEKQIKHFGMLRRWDDSQKYLSDNVHLVCEETANYLVIWCIDLEVEEKCALMEQVAHQTIVMQFILELAKSLKVDPRACFRQFFTKIKTADRQYMEGFNDELEAFKERVRGRAKLRIEKAMKEYEEEERKKRLGPGGLDPVEVYESLPEELQKCFDVKDVQMLQDAISKMDPTDAKYHMQRCIDSGLWVPNSKASEAKEGEEAGPGDPLLEAVPKTGDEKDVSV

SEQ ID NO: 46 - protein, 321 aa, synthetic construct
  REGION 1..321: note = Synthetic Polypeptide
MEMEKEFEQIDKSGSWAAIYQDIRHEASDFPCRVAKLPKNKNRNRYRDVSPFDHSRIKLHQEDNDYINASLIKMEEAQRSYILTQGPLPNTCGHFWEMVWEQKSRGVVMLNRVMEKGSLKCAQYWPQKEEKEMIFEDTNLKLTLISEDIKSYYTVRQLELENLTTQETREILHFHYTTWPDFGVPESPASFLNFLFKVRESGSLSPEHGPVVVHSSAGIGRSGTFCLADTCLLLMDKRKDPSSVDIKKVLLEMRKFRMGLIQTADQLRFSYLAVIEGAKFIMGDSSVQDQWKELSHEDLEPPPEHIPPPPRPPKRILEPHN

SEQ ID NO: 47 - protein, 371 aa, synthetic construct
  REGION 1..371: note = Synthetic Polypeptide
MKIEEGKLVIWINGDKGYNGLAEVGKKFEKDTGIKVTVEHPDKLEEKFPQVAATGDGPDIIFWAHDRFGGYAQSGLLAEITPDKAFQDKLYPFTWDAVRYNGKLIAYPIAVEALSLIYNKDLLPNPPKTWEEIPALDKELKAKGKSALMFNLQEPYFTWPLIAADGGYAFKYENGKYDIKDVGVDNAGAKAGLTFLVDLIKNKHMNADTDYSIAEAAFNKGETAMTINGPWAWSNIDTSKVNYGVTVLPTFKGQPSKPFVGVLSAGINAASPNKELAKEFLENYLLTDEGLEAVNKDKPLGAVALKSYEEELAKDPRIAATMENAQKGEIMPNIPQMSAFWYAVRTAVINAASGRQTVDEALKDAQTRITK

SEQ ID NO: 48 - protein, 707 aa, synthetic construct
  REGION 1..707: note = Synthetic Polypeptide
MKFGNFLLTYQPPQFSQTEVMKRLVKLGRISEECGFDTVWLLEHHFTEFGLLGNPYVAAAYLLGATKKLNVGTAAIVLPTAHPVRQLEDVNLLDQMSKGRFRFGICRGLYNKDFRVFGTDMNNSRALAECWYGLIKNGMTEGYMEADNEHIKFHKVKVNPAAYSRGGAPVYVVAESASTTEWAAQFGLPMILSWIINTNEKKAQLELYNEVAQEYGHDIHNIDHCLSYITSVDHDSIKAKEICRKFLGHWYDSYVNATTIFDDSDQTRGYDFNKGQWRDFVLKGHKDTNRRIDYSYEINPVGTPQECIDIIQKDIDATGISNICCGFEANGTVDEIIASMKLFQSDVMPFLKEKQRSLLYYGGGGSGGGGSGGGGSGGGGSKFGLFFLNFINSTTVQEQSIVRMQEITEYVDKLNFEQILVYENHFSDNGVVGAPLTVSGFLLGLTEKIKIGSLNHIITTHHPVRIAEEACLLDQLSEGRFILGFSDCEKKDEMHFFNRPVEYQQQLFEECYEIINDALTTGYCNPDNDFYSFPKISVNPHAYTPGGPRKYVTATSHHIVEWAAKKGIPLIFKWDDSNDVRYEYAERYKAVADKYDVDLSEIDHQLMILVNYNEDSNKAKQETRAFISDYVLEMHPNENFENKLEEIIAENAVGNYTECITAAKLAIEKCGAKSVLLSFEPMNDLMSQKNVINIVDDNIKKYHTEYT

SEQ ID NO: 49 - protein, 263 aa, synthetic construct
  REGION 1..263: note = Synthetic Polypeptide
MREAVIAEVSTQLSEVVGVIERHLEPTLLAVHLYGSAVDGGLKPHSDIDLLVTVTVRLDETTRRALINDLLETSASPGESEILRAVEVTIVVHDDIIPWRYPAKRELQFGEWQRNDILAGIFEPATIDIDLAILLTKAREHSVALVGPAAEELFDPVPEQDLFEALNETLTLWNSPPDWAGDERNVVLTLSRIWYSAVTGKIAPKDVAADWAMERLPAQYQPVILEARQAYLGQEEDRLASRADQLEEFVHYVKGEITKVVGK

SEQ ID NO: 50 - protein, 785 aa, synthetic construct
  REGION 1..785: note = Synthetic Polypeptide
MVKREFPPGFWKDDLIDSLTSSHKVAASDEKRIETLISEIKNMFRCMGYGETNPSAYDTAWVARIPAVDGSDNPHFPETVEWILQNQLKDGSWGEGFYFLAYDRILATLACIITLTLWRTGETQVQKGIEFFRTQAGKMEDEADSHRPSGFEIVFPAMLKEAKILGLDLPYDLPFLKQIIEKREAKLKRIPTDVLYALPTTLLYSLEGLQEIVDWQKIMKLQSKDGSFLSSPASTAAVFMRTGNKKCLDFLNFVLKKFGNHVPCHYPLDLFERLWAVDTVERLGIDRHFKEEIKEALDYVYSHWDERGIGWARENPVPDIDDTAMGLRILRLHGYNVSSDVLKTFRDENGEFFCFLGQTQRGVTDMLNVNRCSHVSFPGETIMEEAKLCTERYLRNALENVDAFDKWAFKKNIRGEVEYALKYPWHKSMPRLEARSYIENYGPDDVWLGKTVYMMPYISNEKYLELAKLDFNKVQSIHQTELQDLRRWWKSSGFTDLNFTRERVTEIYFSPASFIFEPEFSKCREVYTKTSNFTVILDDLYDAHGSLDDLKLFTESVKRWDLSLVDQMPQQMKICFVGFYNTFNDIAKEGRERQGRDVLGYIQNVWKVQLEAYTKEAEWSEAKYVPSFNEYIENASVSIALGTVVLISALFTGEVLTDEVLSKIDRESRFLQLMGLTGRLVNDTKTYQAERGQGEVASAIQCYMKDHPKISEEEALQHVYSVMENALEELNREFVNNKIPDIYKRLVFETARIMQLFYMQGDGLTLSHDMEIKEHVKNCLFQPVA

SEQ ID NO: 51 - protein, 296 aa, synthetic construct
  REGION 1..296: note = Synthetic Polypeptide
MFDFNEYMKSKAVAVDAALDKAIPLEYPEKIHESMRYSLLAGGKRVRPALCIAACELVGGSQDLAMPTACAMEMIHTMSLIHDDLPCMDNDDFRRGKPTNHKVFGEDTAVLAGDALLSFAFEHIAVATSKTVPSDRTLRVISELGKTIGSQGLVGGQVVDITSEGDANVDLKTLEWIHIHKTAVLLECSVVSGGILGGATEDEIARIRRYARCVGLLFQVVDDILDVTKSSEELGKTAGKDLLTDKATYPKLMGLEKAKEFAAELATRAKEELSSFDQIKAAPLLGLADYIAFRQN

SEQ ID NO: 52 - protein, 1049 aa, synthetic construct [sequence omitted]

SEQ ID NO: 53 - protein, 142 aa, synthetic construct
  REGION 1..142: note = Synthetic Polypeptide
AATLERIEKNFVITDPRLPDNPIIFASDSFLQLTEYSREEILGRNCRFLQGPETDRATVRKIRDAIDNQTEVTVQLINYTKSGKKFWNLFHLQPMRDQKGDVQYFIGVQLDGTEHVRDAAEREGVMLIKKTAENIDEAAKEL

SEQ ID NO: 54 - protein, 748 aa, synthetic construct
  REGION 1..748: note = Synthetic Polypeptide
MASVAGHASGSPAFGTADLSNCEREEIHLAGSIQPHGALLVVSEPDHRIIQASANAAEFLNLGSVLGVPLAEIDGDLLIKILPHLDPTAEGMPVAVRCRIGNPSTEYDGLMHRPPEGGLIIELERAGPPIDLSGTLAPALERIRTAGSLRALCDDTALLFQQCTGYDRVMVYRFDEQGHGEVFSERHVPGLESYFGNRYPSSDIPQMARRLYERQRVRVLVDVSYQPVPLEPRLSPLTGRDLDMSGCFLRSMSPIHLQYLKNMGVRATLVVSLVVGGKLWGLVACHHYLPRFMHFELRAICELLAEAIATRITALESFAQSQSELFVQRLEQRMIEAITREGDWRAAIFDTSQSILQPLHAAGCALVYEDQIRTIGDVPSTQDVREIAGWLDRQPRAAVTSTASLGLDVPELAHLTRMASGVVAAPISDHRGEFLMWFRPERVHTVTWGGDPKKPFTMGDTPADLSPRRSFAKWHQVVEGTSDPWTAADLAAARTIGQTVADIVLQFRAVRTLIAREQYEQFSSQVHASMQPVLITDAEGRILLMNDSFRDMLPAGSPSAVHLDDLAGFFVESNDFLRNVAELIDHGRGWRGEVLLRGAGNRPLPLAVRADPVTRTEDQSLGFVLIFSDATDRRTADAARTRFQEGILASARPGVRLDSKSDLLHEKLLSALVENAQLAALEITYGVETGRIAELLEGVRQSMLRTAEVLGHLVQHAARTAGSDSSSNGSQNKKEFDSAGSAGSAGTS

SEQ ID NO: 55 - protein, 295 aa, synthetic construct
  REGION 1..295: note = Synthetic Polypeptide
MGMPTTIEREFEELDTQRRWQPLYLEIRNESHDYPHRVAKFPENRNRNRYRDVSPYDHSRVKLQNAENDYINASLVDIEEAQRSYILTQGPLPNTCCHFWLMVWQQKTKAVVMLNRIVEKESVKCAQYWPTDDQEMLFKETGFSVKLLSEDVKSYYTVHLLQLENINSGETRTISHFHYTTWPDFGVPESPASFLNFLFKVRESGSLNPDHGPAVIHCSAGIGRSGTFSLVDTCLVLMEKGDDINIKQVLLNMRKYRMGLIQTPDQLRFSYMAIIEGAKCIKGDSSIQKRWKELS

SEQ ID NO: 56 - protein, 435 aa, synthetic construct
  REGION 1..435: note = Synthetic Polypeptide
MEMEKEFEQIDKSGSWAAIYQDIRHEASDFPCRVAKLPKNKNRNRYRDVSPFDHSRIKLHQEDNDYINASLIKMEEAQRSYILTQGPLPNTCGHFWEMVWEQKSRGVVMLNRVMEKGSLKCAQYWPQKEEKEMIFEDTNLKLTLISEDIKSYYTVRQLELENLTTQETREILHFHYTTWPDFGVPESPASFLNFLFKVRESGSLSPEHGPVVVHCSAGIGRSGTFCLADTCLLLMDKRKDPSSVDIKKVLLEMRKFRMGLIQTADQLRFSYLAVIEGAKFIMGDSSVQDQWKELSHEDLEPPPEHIPPPPRPPKRILEPHNGKCREFFPNHQWVKEETQEDKDCPIKEEKGSPLNAAPYGIESMSQDTEVRSRVVGGSLRGAQAASPAKGEPSLPEKDEDHALSYWKPFLVNMCVATVLTAGAYLCYRFLFNSNT

SEQ ID NO: 57 - protein, 473 aa, synthetic construct
  REGION 1..473: note = Synthetic Polypeptide
MNIKKFAKQATVLTFTTALLAGGATQAFAKETNQKPYKETYGISHITRHDMLQIPEQQKNEKYQVPEFDSSTIKNISSAKGLDVWDSWPLQNADGTVANYHGYHIVFALAGDPKNADDTSIYMFYQKVGETSIDSWKNAGRVFKDSDKFDANDSILKDQTQEWSGSATFTSDGKIRLFYTDFSGKHYGKQTLTTAQVNVSASDSSLNINGVEDYKSIFDGDGKTYQNVQQFIDEGNYSSGDNHTLRDPHYVEDKGHKYLVFEANTGTEDGYQGEESLFNKAYYGKSTSFFRQESQKLLQSDKKRTAELANGALGMIELNDDYTLKKVMKPLIASNTVTDEIERANVFKMNGKWYLFTDSRGSKMTIDGITSNDIYMLGYVSNSLTGPYKPLNKTGLVLKMDLDPNDVTFTYSHFAVPQAKGNNVVITSYMTNRGFYADKQSTFAPSFLLNIKGKKTSVVKDSILEQGQLTVNK

SEQ ID NO: 58 - protein, 382 aa, synthetic construct
  REGION 1..382: note = Synthetic Polypeptide
MSLKEKTQSLFANAFGYPATHTIQAPGRVNLIGEHTDYNDGFVLPCAIDYQTVISCAPRDDRKVRVMAADYENQLDEFSLDAPIVAHENYQWANYVRGVVKHLQLRNNSFGGVDMVISGNVPQGAGLSSSASLEVAVGTVLQQLYHLPLDGAQIALNGQEAENQFVGCNCGIMDQLISALGKKDHALLIDCRSLGTKAVSMPKGVAVVIINSNFKRTLVGSEYNTRREQCETGARFFQQPALRDVTIEEFNAVAHELDPIVAKRVRHILTENARTVEAASALEQGDLKRMGELMAESHASMRDDFEITVPQIDTLVEIVKAVIGDKGGVRMTGGGFGGCIVALIPEELVPAVQQAVAEQYEAKTGIKETFYVCKPSQGAGQC

SEQ ID NO: 59 - protein, 593 aa, synthetic construct
  REGION 1..593: note = Synthetic Polypeptide
MAQISESVSPSTDLKSTESSITSNRHGNMWEDDRIQSLNSPYGAPAYQERSEKLIEEIKLLFLSDMDDSCNDSDRDLIKRLEIVDTVECLGIDRHFQPEIKLALDYVYRCWNERGIGEGSRDSLKKDLNATALGFRALRLHRYNVSSGVLENFRDDNGQFFCGSTVEEEGAEAYNKHVRCMLSLSRASNILFPGEKVMEEAKAFTTNYLKKVLAGREATHVDESLLGEVKYALEFPWHCSVQRWEARSFIEIFGQIDSELKSNLSKKMLELAKLDFNILQCTHQKELQIISRWFADSSIASLNFYRKCYVEFYFWMAAAISEPEFSGSRVAFTKIAILMTMLDDLYDTHGTLDQLKIFTEGVRRWDVSLVEGLPDFMKIAFEFWLKTSNELIAEAVKAQGQDMAAYIRKNAWERYLEAYLQDAEWIATGHVPTFDEYLNNGTPNTGMCVLNLIPLLLMGEHLPIDILEQIFLPSRFHHLIELASRLVDDARDFQAEKDHGDLSCIECYLKDHPESTVEDALNHVNGLLGNCLLEMNWKFLKKQDSVPLSCKKYSFHVLARSIQFMYNQGDGFSISNKVIKDQVQKVLIVPVPI

SEQ ID NO: 60 - protein, 546 aa, synthetic construct
  REGION 1..546: note = Synthetic Polypeptide
MALTEEKPIRPIANFPPSIWGDQFLIYEKQVEQGVEQIVNDLKKEVRQLLKEALDIPMKHANLLKLIDEIQRLGIPYHFEREIDHALQCIYETYGDNWNGDRSSLWFRLMRKQGYYVTCDVFNNYKDKNGAFKQSLANDVEGLLELYEATSMRVPGEIILEDALGFTRSRLSIMTKDAFSTNPALFTEIQRALKQPLWKRLPRIEAAQYIPFYQQQDSHNKTLLKLAKLEFNLLQSLHKEELSHVCKWWKAFDIKKNAPCLRDRIVECYFWGLGSGYEPQYSRARVFFTKAVAVITLIDDTYDAYGTYEELKIFTEAVERWSITCLDTLPEYMKPIYKLFMDTYTEMEEFLAKEGRTDLFNCGKEFVKEFVRNLMVEAKWANEGHIPTTEEHDPVVIITGGANLLTTTCYLGMSDIFTKESVEWAVSAPPLFRYSGILGRRLNDLMTHKAEQERKHSSSSLESYMKEYNVNEEYAQTLIYKEVEDVWKDINREYLTTKNIPRPLLMAVIYLCQFLEVQYAGKDNFTRMGDEYKHLIKSLLVYPMSI

SEQ ID NO: 61 - protein, 802 aa, synthetic construct
  REGION 1..802: note = Synthetic Polypeptide
MSSSTGTSKVVSETSSTIVDDIPRLSANYHGDLWHHNVIQTLETPFRESSTYQERADELVVKIKDMFNALGDGDISPSAYDTAWVARLATISSDGSEKPRFPQALNWVFNNQLQDGSWGIESHFSLCDRLLNTTNSVIALSVWKTGHSQVQQGAEFIAENLRLLNEEDELSPDFQIIFPALLQKAKALGINLPYDLPFIKYLSTTREARLTDVSAAADNIPANMLNALEGLEEVIDWNKIMRFQSKDGSFLSSPASTACVLMNTGDEKCFTFLNNLLDKFGGCVPCMYSIDLLERLSLVDNIEHLGIGRHFKQEIKGALDYVYRHWSERGIGWGRDSLVPDLNTTALGLRTLRMHGYNVSSDVLNNFKDENGRFFSSAGQTHVELRSVVNLFRASDLAFPDERAMDDARKFAEPYLREALATKISTNTKLFKEIEYVVEYPWHMSIPRLEARSYIDSYDDNYVWQRKTLYRMPSLSNSKCLELAKLDFNIVQSLHQEELKLLTRWWKESGMADINFTRHRVAEVYFSSATFEPEYSATRIAFTKIGCLQVLFDDMADIFATLDELKSFTEGVKRWDTSLLHEIPECMQTCFKVWFKLMEEVNNDVVKVQGRDMLAHIRKPWELYFNCYVQEREWLEAGYIPTFEEYLKTYAISVGLGPCTLQPILLMGELVKDDVVEKVHYPSNMFELVSLSWRLTNDTKTYQAEKARGQQASGIACYMKDNPGATEEDAIKHICRVVDRALKEASFEYFKPSNDIPMGCKSFIFNLRLCVQIFYKFIDGYGIANEEIKDYIRKVYIDPIQV

SEQ ID NO: 62 - protein, 317 aa, synthetic construct
  REGION 1..317: note = Synthetic Polypeptide
MPTTIEREFEELDTQRRWQPLYLEIRNESHDYPHRVAKFPENRNRNRYRDVSPYDHSRVKLQNAENDYINASLVDIEEAQRSYILTQGPLPNTCCHFWLMVWQQKTKAVVMLNRIVEKESVKCAQYWPTDDQEMLFKETGFSVKLLSEDVKSYYTVHLLQLENINSGETRTISHFHYTTWPDFGVPESPASFLNFLFKVRESGSLNPDHGPAVIHCSAGIGRSGTFSLVDTCLVLMEKGDDINIKQVLLNMRKYRMGLIQTPDQLRFSYMAIIEGAKCIKGDSSIQKRWKELSKEDLSPAFDHSPNKIMTEKYNGNR

SEQ ID NO: 63 - protein, 299 aa, synthetic construct
  REGION 1..299: note = Synthetic Polypeptide
MSSGVDLGTENLYFQSMSRVLQAEELHEKALDPFLLQAEFFEIPMNFVDPKEYDIPGLVRKNRYKTILPNPHSRVCLTSPDPDDPLSSYINANYIRGYGGEEKVYIATQGPIVSTVADFWRMVWQEHTPIIVMITNIEEMNEKCTEYWPEEQVAYDGVEITVQKVIHTEDYRLRLISLKSGTEERGLKHYWFTSWPDQKTPDRAPPLLHLVREVEEAAQQEGPHCAPIIVHCSAGIGRTGCFIATSICCQQLRQEGVVDILKTTCQLRQDRGGMIQTCEQYQFVHHVMSLYEKQLSHQS

SEQ ID NO: 64 - protein, 595 aa, synthetic construct [sequence omitted]

SEQ ID NO: 65 - protein, 593 aa, synthetic construct [sequence omitted]

SEQ ID NO: 66 - protein, 425 aa, synthetic construct
  REGION 1..425: note = Synthetic Polypeptide
MEQVEILRKFIQRVQAMKSPDHNGEDNFARDFMRLRRLSTKYRTEKIYPTATGEKEENVKKNRYKDILPFDHSRVKLTLKTPSQDSDYINANFIKGVYGPKAYVATQGPLANTVIDFWRMVWEYNVVIIVMACREFEMGRKKCERYWPLYGEDPITFAPFKISCEDEQARTDYFIRTLLLEFQNESRRLYQFHYVNWPDHDVPSSFDSILDMISLMRKYQEHEDVPICIHCSAGCGRTGAICAIDYTWNLLKAGKIPEEFNVFNLIQEMRTQRHSAVQTKEQYELVHRAIAQLFEKQLQLYEIHGAQKIADGVNEINTENMVSSIEPEKQDSPPPKPPRTRSCLVEGDAKEEILQPPEPHPVPPILTPSPPSAFPTVTTVWQDNDRYHPKPVLQWFHQNNIQQTSTETIVNQQNFQGKMNQQLNR

SEQ ID NO: 67 - protein, 299 aa, synthetic construct
  REGION 1..299: note = Synthetic Polypeptide
MDQREILQKFLDEAQSKKITKEEFANEFLKLKRQSTKYKADKTYPTTVAEKPKNIKKNRYKDILPYDYSRVELSLITSDEDSSYINANFIKGVYGPKAYIATQGPLSTTLLDFWRMIWEYSVLIIVMACMEYEMGKKKCERYWAEPGEMQLEFGPFSVSCEAEKRKSDYIIRTLKVKFNSETRTIYQFHYKNWPDHDVPSSIDPILELIWDVRCYQEDDSVPICIHCSAGCGRTGVICAIDYTWMLLKDGIIPENFSVFSLIREMRTQRPSLVQTQEQYELVYNAVLELFKRQMDVIRD

SEQ ID NO: 68 - protein, 238 aa, synthetic construct
  REGION 1..238: note = Synthetic Polypeptide
MRKGEELFTGVVPILVELDGDVNGHKFSVRGEGEGDATNGKLTLKFICTTGKLPVPWPTLVTTLTYGVQCFARYPDHMKQHDFFKSAMPEGYVQERTISFKDDGTYKTRAEVKFEGDTLVNRIELKGIDFKEDGNILGHKLEYNFNSHNVYITADKQKNGIKANFKIRHNVEDGSVQLADHYQQNTPIGDGPVLLPDNHYLSTQSVLSKDPNEKRDHMVLLEFVTAAGITHGMDELYK

SEQ ID NO: 69 - protein, 245 aa, synthetic construct
  REGION 1..245: note = Synthetic Polypeptide
MHHHHHHVSKGEELFTGVVPILVELDGDVNGHKFSVRGEGEGDATNGKLTLKFICTTGKLPVPWPTLVTTFGYGVACFSRYPDHMKQHDFFKSAMPEGYVQERTISFKDDGTYKTRAEVKFEGDTLVNRIELKGIDFKEDGNILGHKLEYNFNSHNVYITADKQKNGIKANFKIRHNVEDGSVQLADHYQQNTPIGDGPVLLPDNHYLSHQSALSKDPNEKRDHMVLLEFVTAAGITHGMDELYK

SEQ ID NO: 70 - DNA, 129 bp, synthetic construct
  misc_feature 1..129: note = Synthetic Polynucleotide
  source 1..129: mol_type = other DNA
atccggatatagttcctcctttcagcaaaaaacccctcaagacccgtttagaggccccaaggggttatgctagttattgctcagcggtggcagcagccaactcagcttcctttcgggctttgttagcag

SEQ ID NO: 71 - DNA, 426 bp, synthetic construct
  misc_feature 1..426: note = Synthetic Polynucleotide
  source 1..426: mol_type = other DNA
ggctgttttggcggatgagagaagattttcagcctgatacagattaaatcagaacgcagaagcggtctgataaaacagaatttgcctggcggcagtagcgcggtggtcccacctgaccccatgccgaactcagaagtgaaacgccgtagcgccgatggtagtgtggggtcaccccatgcgagagtagggaactgccaggcatcaaataaaacgaaaggctcagtcgaaagactgggcctttcgttttatctgttgtttgtcggtgaacgctctcctgagtaggacaaatccgccgggagcggatttgaacgttgcgaagcaacggcccggagggtggcgggcaggacgcccgccataaactgccaggcatcaaattaagcagaaggccatcctgacggatggcctttttgcgtttctacaaactct

SEQ ID NO: 72 - DNA, 158 bp, synthetic construct
  misc_feature 1..158: note = Synthetic Polynucleotide
  source 1..158: mol_type = other DNA
tgcctggcggcagtagcgcggtggtcccacctgaccccatgccgaactcagaagtgaaacgccgtagcgccgatggtagtgtggggtctccccatgcgagagtagggaactgccaggcatcaaataaaacgaaaggctcagtcgaaagactgggcctt

SEQ ID NO: 73 - DNA, 867 bp, synthetic construct
  misc_feature 1..867: note = Synthetic Polynucleotide
  source 1..867: mol_type = other DNA
atgggctccaagccgcagactcagggcctggccaaggatgcctgggagatccctcgggagtcgctgcggctggaggtcaagctgggccagggctgctttggcgaggtgtggatggggacctggaacggtaccaccagggtggccatcaaaaccctgaagcctggcacgatgtctccagaggccttcctgcaggaggcccaggtcatgaagaagctgaggcatgagaagctggtgcagttgtatgctgtggtttcagaggagcccatttacatcgtcacggagtacatgagcaaggggagtttgctggactttctcaagggggagacaggcaagtacctgcggctgcctcagctggtggacatggctgctcagatcgcctcaggcatggcgtacgtggagcggatgaactacgtccaccgggaccttcgtgcagccaacatcctggtgggagagaacctggtgtgcaaagtggccgactttgggctggctcggctcattgaagacaatgagtacacggcgcggcaaggtgccaaattccccatcaagtggacggctccagaagctgccctctatggccgcttcaccatcaagtcggacgtgtggtccttcgggatcctgctgactgagctcaccacaaagggacgggtgccctaccctgggatggtgaaccgcgaggtgctggaccaggtggagcggggctaccggatgccctgcccgccggagtgtcccgagtccctgcacgacctcatgtgccagtgctggcggaaggagcctgaggagcggcccaccttcgagtacctgcaggccttcctggaggactacttcacgtccaccgagccccagtaccagcccggggagaacctctaa

SEQ ID NO: 74 - DNA, 1137 bp, synthetic construct
  misc_feature 1..1137: note = Synthetic Polynucleotide
  source 1..1137: mol_type = other DNA
atggtggactacagcgtgtgggaccacattgaggtgtctgatgatgaagacgagacgcaccccaacatcgacacggccagtctcttccgctggcggcatcaggcccgggtggaacgcatggagcagttccagaaggagaaggaggaactggacaggggctgccgcgagtgcaagcgcaaggtggccgagtgccagaggaaactgaaggagctggaggtggccgagggcggcaaggcagagctggagcgcctgcaggccgaggcacagcagctgcgcaaggaggagcggagctgggagcagaagctggaggagatgcgcaagaaggagaagagcatgccctggaacgtggacacgctcagcaaagacggcttcagcaagagcatggtaaataccaagcccgagaagacggaggaggactcagaggaggtgagggagcagaaacacaagaccttcgtggaaaaatacgagaaacagatcaagcactttggcatgcttcgccgctgggatgacagccaaaagtacctgtcagacaacgtccacctggtgtgcgaggagacagccaattacctggtcatttggtgcattgacctagaggtggaggagaaatgtgcactcatggagcaggtggcccaccagacaatcgtcatgcaatttatcctggagctggccaagagcctaaaggtggacccccgggcctgcttccggcagttcttcactaagattaagacagccgatcgccagtacatggagggcttcaacgacgagctggaagccttcaaggagcgtgtgcggggccgtgccaagctgcgcatcgagaaggccatgaaggagtacgaggaggaggagcgcaagaagcggctcggccccggcggcctggaccccgtcgaggtctacgagtccctccctgaggaactccagaagtgcttcgatgtgaaggacgtgcagatgctgcaggacgccatcagcaagatggaccccaccgacgcaaagtaccacatgcagcgctgcattgactctggcctctgggtccccaactctaaggccagcgaggccaaggagggagaggaggcaggtcctggggacccattactggaagctgttcccaagacgggcgatgagaaggatgtcagtgtgtaa

SEQ ID NO: 75 - DNA, 1308 bp, synthetic construct
  misc_feature 1..1308: note = Synthetic Polynucleotide
  source 1..1308: mol_type = other DNA
atggagatggaaaaggagttcgagcagatcgacaagtccgggagctgggcggccatttaccaggatatccgacatgaagccagtgacttcccatgtagagtggccaagcttcctaagaacaaaaaccgaaataggtacagagacgtcagtccctttgaccatagtcggattaaactacatcaagaagataatgactatatcaacgctagtttgataaaaatggaagaagcccaaaggagttacattcttacccagggccctttgcctaacacatgcggtcacttttgggagatggtgtgggagcagaaaagcaggggtgtcgtcatgctcaacagagtgatggagaaaggttcgttaaaatgcgcacaatactggccacaaaaagaagaaaaagagatgatctttgaagacacaaatttgaaattaacattgatctctgaagatatcaagtcatattatacagtgcgacagctagaattggaaaaccttacaacccaagaaactcgagagatcttacatttccactataccacatggcctgactttggagtccctgaatcaccagcctcattcttgaactttcttttcaaagtccgagagtcagggtcactcagcccggagcacgggcccgttgtggtgcactgcagtgcaggcatcggcaggtctggaaccttctgtctggctgatacctgcctcttgctgatggacaagaggaaagacccttcttccgttgatatcaagaaagtgctgttagaaatgaggaagtttcggatggggctgatccagacagccgaccagctgcgcttctcctacctggctgtgatcgaaggtgccaaattcatcatgggggactcttccgtgcaggatcagtggaaggagctttcccacgaggacctggagcccccacccgagcatatccccccacctccccggccacccaaacgaatcctggagccacacaatgggaaatgcagggagttcttcccaaatcaccagtgggtgaaggaagagacccaggaggataaagactgccccatcaaggaagaaaaaggaagccccttaaatgccgcaccctacggcatcgaaagcatgagtcaagacactgaagttagaagtcgggtcgtggggggaagtcttcgaggtgcccaggctgcctccccagccaaaggggagccgtcactgcccgagaaggacgaggaccatgcactgagttactggaagcccttcctggtcaacatgtgcgtggctacggtcctcacggccggcgcttacctctgctacaggttcctgttcaacagcaacacatag

SEQ ID NO: 76 - DNA, 1086 bp, synthetic construct
  misc_feature 1..1086: note = Synthetic Polynucleotide
  source 1..1086: mol_type = other DNA
atgaaatttggaaactttttgcttacataccaacctccccaattttcccaaacagaggtaatgaaacgtttggttaaattaggtcgcatctctgaggagtgtggttttgataccgtatggttactggagcatcatttcacggagtttggtttgcttggtaacccttatgtcgctgctgcatatttacttggcgcgactaaaaaattgaatgtaggaactgccgctattgttcttcccacagcccatccagtacgccaacttgaagatgtgaatttattggatcaaatgtcaaaaggacgatttcggtttggtatttgccgagggctttacaacaaggactttcgcgtattcggcacagatatgaataacagtcgcgccttagcggaatgctggtacgggctgataaagaatggcatgacagagggatatatggaagctgataatgaacatatcaagttccataaggtaaaagtaaaccccgcggcgtatagcagaggtggcgcaccggtttatgtggtggctgaatcagcttcgacgactgagtgggctgctcaatttggcctaccgatgatattaagttggattataaatactaacgaaaagaaagcacaacttgagctttataatgaagtggctcaagaatatgggcacgatattcataatatcgaccattgcttatcatatataacatctgtagatcatgactcaattaaagcgaaagagatttgccggaaatttctggggcattggtatgattcttatgtgaatgctacgactatttttgatgattcagaccaaacaagaggttatgatttcaataaagggcagtggcgtgactttgtattaaaaggacataaagatactaatcgccgtattgattacagttacgaaatcaatcccgtgggaacgccgcaggaatgtattgacataattcaaaaagacattgatgctacaggaatatcaaatatttgttgtggatttgaagctaatggaacagtagacgaaattattgcttccatgaagctcttccagtctgatgtcatgccatttcttaaagaaaaacaacgttcgctattatattattaa

SEQ ID NO: 77 - DNA, 987 bp, synthetic construct
  misc_feature 1..987: note = Synthetic Polynucleotide
  source 1..987: mol_type = other DNA
atgagcaaatttggattgttcttccttaacttcatcaattcaacaactgttcaagaacagagtatagttcgcatgcaggaaataacggagtatgttgataagttgaattttgaacagattttagtgtatgaaaatcatttttcagataatggtgttgtcggcgctcctctgactgtttctggttttctgctcggtttaacagagaaaattaaaattggttcattaaatcacatcattacaactcatcatcctgtccgcatagcggaggaagcttgcttattggatcagttaagtgaagggagatttattttagggtttagtgattgcgaaaaaaaagatgaaatgcatttttttaatcgcccggttgaatatcaacagcaactatttgaagagtgttatgaaatcattaacgatgctttaacaacaggctattgtaatccagataacgatttttatagcttccctaaaatatctgtaaatccccatgcttatacgccaggcggacctcggaaatatgtaacagcaaccagtcatcatattgttgagtgggcggccaaaaaaggtattcctctcatctttaagtgggatgattctaatgatgttagatatgaatatgctgaaagatataaagccgttgcggataaatatgacgttgacctatcagagatagaccatcagttaatgatattagttaactataacgaagatagtaataaagctaaacaagaaacgcgtgcatttattagtgattatgttcttgaaatgcaccctaatgaaaatttcgaaaataaacttgaagaaataattgcagaaaacgctgtcggaaattatacggagtgtataactgcggctaagttggcaattgaaaagtgtggtgcgaaaagtgtattgctgtcctttgaaccaatgaatgatttgatgagccaaaaaaatgtaatcaatattgttgatgataatattaagaagtaccacacggaatatacctaa

SEQ ID NO: 78 - DNA, 276 bp, synthetic construct
  misc_feature 1..276: note = Synthetic Polynucleotide
  source 1..276: mol_type = other DNA
atggcacgcgtaactgttcaggacgctgtagagaaaattggtaaccgttttgacctggtactggtcgccgcgcgtcgcgctcgtcagatgcaggtaggcggaaaggatccgctggtaccggaagaaaacgataaaaccactgtaatcgcgctgcgcgaaatcgaagaaggtctgatcaacaaccagatcctcgacgttcgcgaacgccaggaacagcaagagcaggaagccgctgaattacaagccgttaccgctattgctgaaggtcgtcgttaa

SEQ ID NO: 79 - DNA, 636 bp, synthetic construct
  misc_feature 1..636: note = Synthetic Polynucleotide
  source 1..636: mol_type = other DNA
atgagtatcagcagcagggtaaaaagcaaaagaattcagcttggacttaaccaggctgaacttgctcaaaaggtggggactacccagcagtctatagagcagctcgaaaacggtaaaactaagcgaccacgctttttaccagaacttgcgtcagctcttggcgtaagtgttgactggctgctcaatggcacctctgattcgaatgttagatttgttgggcacgttgagcccaaagggaaatatccattgattagcatggttagagctcgttcgtggtgtgaagcttgtgaaccctacgatatcaaggacattgatgaatggtatgacagtgacgttaacttattaggcaatggattctggctgaaggttgaaggtgattccatgacctcacctgtaggtcaaagcatccctgaaggtcatatggtgttagtagatactggacgggagccagtgaatggaagccttgttgtagccaaactgactgacgcgaacgaagcaacattcaagaaactggtcatagatggcggtcagaagtacctgaaaggcctgaatccttcatggcctatgactcctatcaacggaaactgcaagattatcggtgttgtcgtggaagcgagggtaaaattcgtagactaa

SEQ ID NO: 80 - DNA, 300 bp, synthetic construct
  misc_feature 1..300: note = Synthetic Polynucleotide
  source 1..300: mol_type = other DNA
atgtggtattttgggaagatcactcgtcgggagtccgagcggctgctgctcaaccccgaaaacccccggggaaccttcttggtccgggagagcgagacggtaaaaggtgcctatgccctctccgtttctgactttgacaacgccaaggggctcaatgtgaaacactacctgatccgcaagctggacagcggcggcttctacatcacctcacgcacacagttcagcagcctgcagcagctggtggcctactactccaaacatgctgatggcttgtgccaccgcctgaccaacgtctgctaa

SEQ ID NO: 81 - DNA, 1116 bp, synthetic construct
  misc_feature 1..1116: note = Synthetic Polynucleotide
  source 1..1116: mol_type = other DNA
atgaaaatcgaagaaggtaaactggtaatctggattaacggcgataaaggctataacggtctcgctgaagtcggtaagaaattcgagaaagataccggaattaaagtcaccgttgagcatccggataaactggaagagaaattcccacaggttgcggcaactggcgatggccctgacattatcttctgggcacacgaccgctttggtggctacgctcaatctggcctgttggctgaaatcaccccggacaaagcgttccaggacaagctgtatccgtttacctgggatgccgtacgttacaacggcaagctgattgcttacccgatcgctgttgaagcgttatcgctgatttataacaaagatctgctgccgaacccgccaaaaacctgggaagagatcccggcgctggataaagaactgaaagcgaaaggtaagagcgcgctgatgttcaacctgcaagaaccgtacttcacctggccgctgattgctgctgacgggggttatgcgttcaagtatgaaaacggcaagtacgacattaaagacgtgggcgtggataacgctggcgcgaaagcgggtctgaccttcctggttgacctgattaaaaacaaacacatgaatgcagacaccgattactccatcgcagaagctgcctttaataaaggcgaaacagcgatgaccatcaacggcccgtgggcatggtccaacatcgacaccagcaaagtgaattatggtgtaacggtactgccgaccttcaagggtcaaccatccaaaccgttcgttggcgtgctgagcgcaggtattaacgccgccagtccgaacaaagagctggcgaaagagttcctcgaaaactatctgctgactgatgaaggtctggaagcggttaataaagacaaaccgctgggtgccgtagcgctgaagtcttacgaggaagagttggcgaaagatccacgtattgccgccaccatggaaaacgcccagaaaggtgaaatcatgccgaacatcccgcagatgtccgctttctggtatgccgtgcgtactgcggtgatcaacgccgccagcggtcgtcagactgtcgatgaagccctgaaagacgcgcagactcgtatcaccaagtaa

SEQ ID NO: 82 - DNA, 36 bp, synthetic construct
  misc_feature 1..36: note = Synthetic Polynucleotide
  source 1..36: mol_type = other DNA
tggatggaggactatgactacgtccacctacagggg

SEQ ID NO: 83 - DNA, 33 bp, synthetic construct
  misc_feature 1..33: note = Synthetic Polynucleotide
  source 1..33: mol_type = other DNA
gaaccgcagtatgaagaaattccgatttatctg

SEQ ID NO: 84 - DNA, 30 bp, synthetic construct
  misc_feature 1..30: note = Synthetic Polynucleotide
  source 1..30: mol_type = other DNA
ccgcagcgctatctggtgattcagggcgat

SEQ ID NO: 85 - DNA, 30 bp, synthetic construct
  misc_feature 1..30: note = Synthetic Polynucleotide
  source 1..30: mol_type = other DNA
gatcatcagtattataacgattttccgggc

SEQ ID NO: 86 - DNA, 5432 bp, synthetic construct
  misc_feature 1..5432: note = Synthetic Polynucleotide
  misc_feature 1317: note = n is a, c, g, or t
  source 1..5432: mol_type = other DNA
atgtcattaccgttcttaacttctgcaccgggaaaggttattatttttggtgaacactctgctgtgtacaacaagcctgccgtcgctgctagtgtgtctgcgttgagaacctacctgctaataagcgagtcatctgcaccagatactattgaattggacttcccggacattagctttaatcataagtggtccatcaatgatttcaatgccatcaccgaggatcaagtaaactcccaaaaattggccaaggctcaacaagccaccgatggcttgtctcaggaactcgttagtcttttggatccgttgttagctcaactatccgaatccttccactaccatgcagcgttttgtttcctgtatatgtttgtttgcctatgcccccatgccaagaatattaagttttctttaaagtctactttacccatcggtgctgggttgggctcaagcgcctctatttctgtatcactggccttagctatggcctacttgggggggttaataggatctaatgacttggaaaagctgtcagaaaacgataagcatatagtgaatcaatgggccttcataggtgaaaagtgtattcacggtaccccttcaggaatagataacgctgtggccacttatggtaatgccctgctatttgaaaaagactcacataatggaacaataaacacaaacaattttaagttcttagatgatttcccagccattccaatgatcctaacctatactagaattccaaggtctacaaaagatcttgttgctcgcgttcgtgtgttggtcaccgagaaatttcctgaagttatgaagccaattctagatgccatgggtgaatgtgccctacaaggcttagagatcatgactaagttaagtaaatgtaaaggcaccgatgacgaggctgtagaaactaataatgaactgtatgaacaactattggaattgataagaataaatcatggactgcttgtctcaatcggtgtttctcatcctggattagaacttattaaaaatctgagcgatgatttgagaattggctccacaaaacttaccggtgctggtggcggcggttgctctttgactttgttacgaagagacattactcaagagcaaattgacagcttcaaaaagaaattgcaagatgattttagttacgagacatttgaaacagacttgggtgggactggctgctgtttgttaagcgcaaaaaatttgaataaagatcttaaaatcaaatccctagtattccaattatttgaaaataaaactaccacaaagcaacaaattgacgatctattattgccaggaaacacgaatttnccatggacttcataggaggcagatcaaatgtcagagttgagagccttcagtgccccagggaaagcgttactagctggtggatatttagttttagatacaaaatatgaagcatttgtagtcggattatcggcaagaatgcatgctgtagcccatccttacggttcattgcaagggtctgataagtttgaagtgcgtgtgaaaagtaaacaatttaaagatggggagtggctgtaccatataagtcctaaaagtggcttcattcctgtttcgataggcggatctaagaaccctttcattgaaaaagttatcgctaacgtatttagctactttaaacctaacatggacgactactgcaatagaaacttgttcgttattgatattttctctgatgatgcctaccattctcaggaggatagcgttaccgaacatcgtggcaacagaagattgagttttcattcgcacagaattgaagaagttcccaaaacagggctgggctcctcggcaggtttagtcacagttttaactacagctttggcctccttttttgtatcggacctggaaaataatgtagacaaatatagagaagttattcataatttagcacaagttgctcattgtcaagctcagggtaaaattggaagcgggtttgatgtagcggcggcagcatatggatctatcagatatagaagattcccacccgcattaatctctaatttgccagatattggaagtgctacttacggcagtaaactggcgcatttggttgatgaagaagactggaatattacgattaaaagtaaccatttaccttcgggattaactttatggatgggcgatattaagaatggttcagaaacagtaaaactggtccagaaggtaaaaaattggtatgattcgcatatgccagaaagcttgaaaatatatacagaactcgatcatgcaaattctagatttatggatggactatctaaactagatcgcttacacgagactcatgacgattacagcgatcagatatttgagtctcttgagaggaatgactgtacctgtcaaaagtatcctgaaatcacagaagttagagatgcagttgccacaattagacgttcctttagaaaaataactaaagaatctggtgccgatatcgaacctcccgtacaaactagcttattggatgattgccagaccttaaaaggagttcttacttgcttaatacctggtgctggtggttatgacgccattgcagtgattactaagcaagatgttgatcttagggctcaaaccgctaatgacaaaagattttctaaggttcaatggctggatgtaactcaggctgactggggtgttaggaaagaaaaagatccggaaacttatcttgataaataggaggtaatactcatgaccgtttacacagcatccgttaccgcacccgtcaacatcgcaacccttaagtattgggggaaaagggacacgaagttgaatctgcccaccaattcgtccatatcagtgactttatcgcaagatgacctcagaacgttgacctctgcggctactgcacctgagtttgaacgcgacactttgtggttaaatggagaaccacacagcatcgacaatgaaagaactcaaaattgtctgcgcgacctacgccaattaagaaaggaaatggaatcgaaggacgcctcattgcccacattatctcaatggaaactccacattgtctccgaaaataactttcctacagcagctggtttagcttcctccgctgctggctttgctgcattggtctctgcaattgctaagttataccaattaccacagtcaacttcagaaatatctagaatagcaagaaaggggtctggttcagcttgtagatcgttgtttggcggatacgtggcctgggaaatgggaaaagctgaagatggtcatgattccatggcagtacaaatcgcagacagctctgactggcctcagatgaaagcttgtgtcctagttgtcagcgatattaaaaaggatgtgagttccactcagggtatgcaattgaccgtggcaacctccgaactatttaaagaaagaattgaacatgtcgtaccaaagagatttgaagtcatgcgtaaagccattgttgaaaaagatttcgccacctttgcaaaggaaacaatgatggattccaactctttccatgccacatgtttggactctttccctccaatattctacatgaatgacacttccaagcgtatcatcagttggtgccacaccattaatcagttttacggagaaacaatcgttgcatacacgtttgatgcaggtccaaatgctgtgttgtactacttagctgaaaatgagtcgaaactctttgcatttatctataaattgtttggctctgttcctggatgggacaagaaatttactactgagcagcttgaggctttcaaccatcaatttgaatcatctaactttactgcacgtgaattggatcttgagttgcaaaaggatgttgccagagtgattttaactcaagtcggttcaggcccacaagaaacaaacgaatctttgattgacgcaaagactggtctaccaaaggaataactgcagcccgggaggaggattactatatgcaaacggaacacgtcattttattgaatgcacagggagttcccacgggtacgctggaaaagtatgccgcacacacggcagacacccgcttacatctcgcgttctccagttggctgtttaatgccaaaggacaattattagttacccgccgcgcactgagcaaaaaagcatggcctggcgtgtggactaactcggtttgtgggcacccacaactgggagaaagcaacgaagacgcagtgatccgccgttgccgttatgagcttggcgtggaaattacgcctcctgaatctatctatcctgactttcgctaccgcgccaccgatccgagtggcattgtggaaaatgaagtgtgtccggtatttgccgcacgcaccactagtgcgttacagatcaatgatgatgaagtgatggattatcaatggtgtgatttagcagatgtattacacggtattgatgccacgccgtgggcgttcagtccgtggatggtgatgcaggcgacaaatcgcgaagccagaaaacgattatctgcatttacccagcttaaataacccgggggatccactagttctagagcggccgccaccgcggaggaggaatgagtaatggactttccgcagcaactcgaagcctgcgttaagcaggccaaccaggcgctgagccgttttatcgccccactgccctttcagaacactcccgtggtcgaaaccatgcagtatggcgcattattaggtggtaagcgcctgcgacctttcctggtttatgccaccggtcatatgttcggcgttagcacaaacacgctggacgcacccgctgccgccgttgagtgtatccacgcttactcattaattcatgatgatttaccggcaatggatgatgacgatctgcgtcgcggtttgccaacctgccatgtgaagtttggcgaagcaaacgcgattctcgctggcgacgctttacaaacgctggcgttctcgattttaagcgatgccgatatgccggaagtgtcggaccgcgacagaatttcgatgatttctgaactggcgagcgccagtggtattgccggaatgtgcggtggtcaggcattagatttagacgcggaaggcaaacacgtacctctggacgcgcttgagcgtattcatcgtcataaaaccggcgcattgattcgcgccgccgttcgccttggtgcattaagcgccggagataaaggacgtcgtgctctgccggtactcgacaagtatgcagagagcatcggccttgccttccaggttcaggatgacatcctggatgtggtgggagatactgcaacgttgggaaaacgccagggtgccgaccagcaacttggtaaaagtacctaccctgcacttctgggtcttgagcaagcccggaagaaagcccgggatctgatcgacgatgcccgtcagtcgctgaaacaactggctgaacagtcactcgatacctcggcactggaagcgctagcggactacatcatccagcgtaataaataa

SEQ ID NO: 87 - DNA, 1638 bp, synthetic construct
  misc_feature 1..1638: note = Synthetic Polynucleotide
  source 1..1638: mol_type = other DNA
gccctgaccgaagagaaaccgatccgcccgatcgctaacttcccgccgtctatctggggtgaccagttcctgatctacgaaaagcaggttgagcagggtgttgaacagatcgtaaacgacctgaagaaagaagttcgtcagctgctgaaagaagctctggacatcccgatgaaacacgctaacctgttgaagctgatcgacgagatccagcgtctgggtatcccgtaccacttcgaacgcgaaatcgaccacgcactgcagtgcatctacgaaacctacggcgacaactggaacggcgaccgttcttctctgtggtttcgtctgatgcgtaaacagggctactacgttacctgtgacgtttttaacaactacaaggacaagaacggtgctttcaaacagtctctggctaacgacgttgaaggcctgctggaactgtacgaagcgacctccatgcgtgtaccgggtgaaatcatcctggaggacgcgctgggtttcacccgttctcgtctgtccattatgactaaagacgctttctctactaacccggctctgttcaccgaaatccagcgtgctctgaaacagccgctgtggaaacgtctgccgcgtatcgaagcagcacagtacattccgttttaccagcagcaggactctcacaacaagaccctgctgaaactggctaagctggaattcaacctgctgcagtctctgcacaaagaagaactgtctcacgtttgtaagtggtggaaggcatttgacatcaagaaaaacgcgccgtgcctgcgtgaccgtatcgttgaatgttacttctggggtctgggttctggttatgaaccacagtactcccgtgcacgtgtgttcttcactaaagctgtagctgttatcaccctgatcgatgacacttacgatgcttacggcacctacgaagaactgaagatctttactgaagctgtagaacgctggtctatcacttgcctggacactctgccggagtacatgaaaccgatctacaaactgttcatggatacctacaccgaaatggaggaattcctggcaaaagaaggccgtaccgacctgttcaactgcggtaaagagtttgttaaagaattcgtacgtaacctgatggttgaagctaaatgggctaacgaaggccatatcccgactaccgaagaacatgacccggttgttatcatcaccggcggtgcaaacctgctgaccaccacttgctatctgggtatgtccgacatctttaccaaggaatctgttgaatgggctgtttctgcaccgccgctgttccgttactccggtattctgggtcgtcgtctgaacgacctgatgacccacaaagcagagcaggaacgtaaacactcttcctcctctctggaatcctacatgaaggaatataacgttaacgaggagtacgcacagactctgatctataaagaagttgaagacgtatggaaagacatcaaccgtgaatacctgactactaaaaacatcccgcgcccgctgctgatggcagtaatctacctgtgccagttcctggaagtacagtacgctggtaaagataacttcactcgcatgggcgacgaatacaaacacctgatcaaatccctgctggtttacccgatgtccatctga

SEQ ID NO: 88 - DNA, 1782 bp, synthetic construct
  misc_feature 1..1782: note = Synthetic Polynucleotide
  source 1..1782: mol_type = other DNA
atggctcaaatcagcgaatcagtgtctccaagcaccgaccttaaaagcacggaatcttctattaccagcaaccgccacggtaacatgtgggaagatgaccgcattcagagcttaaacagcccatatggcgcacccgcttatcaggaacgtagcgaaaaattgattgaagaaattaagctcctgtttctgtccgatatggacgatagttgcaatgattcggatcgcgacttgatcaaacgcctggagatcgtagatacggttgagtgtctgggcattgatcgtcatttccaacctgaaattaagctggcgctggattacgtgtaccgttgctggaatgagcgtggcatcggagaaggtagccgtgatagcttaaaaaaggacctgaatgcgaccgccttgggctttcgggctttacgcttacaccgttataatgtaagctcaggagtgctggagaacttccgtgatgacaatggtcaattcttttgcggttctactgtggaggaggaaggcgcggaggcctacaataaacatgtacgttgcatgctgtccctgtcccgcgcttccaatattttattcccgggcgagaaagtgatggaagaagcgaaggcgtttacgaccaactatcttaagaaagtcctggcgggtcgtgaagcaactcatgtcgacgagagtctccttggagaggtcaagtatgcactagaatttccgtggcattgttccgtgcagcgctgggaggcacgttcttttatcgaaattttcggtcagattgatagtgaactgaaaagcaacctctctaaaaaaatgctcgaactcgcaaaacttgattttaacatactccagtgtacgcatcaaaaagagctccagatcattagtcgatggttcgccgattcaagtatcgcaagtctgaacttttaccgtaaatgctatgtggaattttacttctggatggccgcggcaatttcagaaccagaatttagtggctctcgcgtggcattcactaaaattgcgatcttgatgacaatgttagatgacttatacgacacgcatgggacgctggatcaattgaaaatatttaccgaaggtgtgcgcaggtgggacgtgtcgctggtggagggcctgccggatttcatgaaaattgcctttgagttctggttaaagacctccaacgaactgattgcggaggcggttaaggcccaaggccaggatatggcggcctatatccgcaaaaacgcttgggaacgctatctggaagcgtatttgcaggatgccgaatggatcgccaccggtcacgttccgacattcgatgaatatctgaacaatggcacccccaacaccggtatgtgtgtacttaatctgatcccgttgctgcttatgggcgaacacttgccgatcgatattcttgaacagatctttctgccgagccggttccaccatctgattgaactggctagccgactggtcgatgatgcgagagattttcaagccgaaaaagatcatggtgatttatcctgcatcgaatgctacctgaaagaccatccggaatcaacagttgaagacgccctgaatcacgtcaacggcctgctggggaattgtttgctggaaatgaattggaaatttctgaaaaaacaggactcggtacctctgtcgtgtaaaaaatactcattccacgtcctggcgcggtcgattcagtttatgtataaccagggggacgggttttcgatttcgaacaaagttattaaagaccaggtccagaaagttctaatcgttccggttcctatataa

SEQ ID NO: 89 - DNA, 2351 bp, synthetic construct
  misc_feature 1..2351: note = Synthetic Polynucleotide
  source 1..2351: mol_type = other DNA
tgaaacgagaatttcctccaggattttggaaggatgatcttatcgattctctaacgtcatctcacaaggttgcagcatcagacgagaagcgtatcgagacattaatatccgagattaagaatatgtttagatgtatgggctatggcgaaacgaatccctctgcatatgacactgcttgggtagcaaggattccagcagttgatggctctgacaaccctcactttcctgagacggttgaatggattcttcaaaatcagttgaaagatgggtcttggggtgaaggattctacttcttggcatatgacagaatactggctacacttgcatgtattattacccttaccctctggcgtactggggagacacaagtacagaaaggtattgaattcttcaggacacaagctggaaagatggaagatgaagctgatagtcataggccaagtggatttgaaatagtatttcctgcaatgctaaaggaagctaaaatcttaggcttggatctgccttacgatttgccattcctgaaacaaatcatcgaaaagcgggaggctaagcttaaaaggattcccactgatgttctctatgcccttccaacaacgttattgtattctttggaaggtttacaagaaatagtagactggcagaaaataatgaaacttcaatccaaggatggatcatttctcagctctccggcatctacagcggctgtattcatgcgtacagggaacaaaaagtgcttggatttcttgaactttgtcttgaagaaattcggaaaccatgtgccttgtcactatccgcttgatctatttgaacgtttgtgggcggttgatacagttgagcggctaggtatcgatcgtcatttcaaagaggagatcaaggaagcattggattatgtttacagccattgggacgaaagaggcattggatgggcgagagagaatcctgttcctgatattgatgatacagccatgggccttcgaatcttgagattacatggatacaatgtatcctcagatgttttaaaaacatttagagatgagaatggggagttcttttgcttcttgggtcaaacacagagaggagttacagacatgttaaacgtcaatcgttgttcacatgtttcatttccgggagaaacgatcatggaagaagcaaaactctgtaccgaaaggtatctgaggaatgctctggaaaatgtggatgcctttgacaaatgggcttttaaaaagaatattcggggagaggtagagtatgcactcaaatatccctggcataagagtatgccaaggttggaggctagaagctatattgaaaactatgggccagatgatgtgtggcttggaaaaactgtatatatgatgccatacatttcgaatgaaaagtatttagaactagcgaaactggacttcaataaggtgcagtctatacaccaaacagagcttcaagatcttcgaaggtggtggaaatcatccggtttcacggatctgaatttcactcgtgagcgtgtgacggaaatatatttctcaccggcatcctttatctttgagcccgagttttctaagtgcagagaggtttatacaaaaacttccaatttcactgttattttagatgatctttatgacgcccatggatctttagacgatcttaagttgttcacagaatcagtcaaaagatgggatctatcactagtggaccaaatgccacaacaaatgaaaatatgttttgtgggtttctacaatacttttaatgatatagcaaaagaaggacgtgagaggcaagggcgcgatgtgctaggctacattcaaaatgtttggaaagtccaacttgaagcttacacgaaagaagcagaatggtctgaagctaaatatgtgccatccttcaatgaatacatagagaatgcgagtgtgtcaatagcattgggaacagtcgttctcattagtgctcttttcactggggaggttcttacagatgaagtactctccaaaattgatcgcgaatctagatttcttcaactcatgggcttaacagggcgtttggtgaatgacaccaaaacttatcaggcagagagaggtcaaggtgaggtggcttctgccatacaatgttatatgaaggaccatcctaaaatctctgaagaagaagctctacaacatgtctatagtgtcatggaaaatgccctcgaagagttgaatagggagtttgtgaataacaaaataccggatatttacaaaagactggtttttgaaactgcaagaataatgcaactcttttatatgcaaggggatggtttgacactatcacatgatatggaaattaaagagcatgtcaaaaattgcctcttccaaccagttgcc

SEQ ID NO: 90 - DNA, 2409 bp, synthetic construct
  misc_feature 1..2409: note = Synthetic Polynucleotide
  source 1..2409: mol_type = other DNA
atgagcagcagcactggcactagcaaggtggtttccgagacttccagtaccattgtggatgatatccctcgactctccgccaattatcatggcgatctgtggcaccacaatgttatacaaactctggagacaccgtttcgtgagagttctacttaccaagaacgggcagatgagctggttgtgaaaattaaagatatgttcaatgcgctcggagacggagatatcagtccgtctgcatacgacactgcgtgggtggcgaggctggcgaccatttcctctgatggatctgagaagccacggtttcctcaggccctcaactgggttttcaacaaccagctccaggatggatcgtggggtatcgaatcgcactttagtttatgcgatcgattgcttaacacgaccaattctgttatcgccctctcggtttggaaaacagggcacagccaagtacaacaaggtgctgagtttattgcagagaatctaagattactcaatgaggaagatgagttgtccccggatttccaaataatctttcctgctctgctgcaaaaggcaaaagcgttggggatcaatcttccttacgatcttccatttatcaaatatttgtcgacaacacgggaagccaggcttacagatgtttctgcggcagcagacaatattccagccaacatgttgaatgcgttggaaggactcgaggaagttattgactggaacaagattatgaggtttcaaagtaaagatggatctttcctgagctcccctgcctccactgcctgtgtactgatgaatacaggggacgaaaaatgtttcacttttctcaacaatctgctcgacaaattcggcggctgcgtgccctgtatgtattccatcgatctgctggaacgcctttcgctggttgataacattgagcatctcggaatcggtcgccatttcaaacaagaaatcaaaggagctcttgattatgtctacagacattggagtgaaaggggcatcggttggggcagagacagccttgttccagatctcaacaccacagccctcggcctgcgaactcttcgcatgcacggatacaatgtttcttcagacgttttgaataatttcaaagatgaaaacgggcggttcttctcctctgcgggccaaacccatgtcgaattgagaagcgtggtgaatcttttcagagcttccgaccttgcatttcctgacgaaagagctatggacgatgctagaaaatttgcagaaccatatcttagagaggcacttgcaacgaaaatctcaaccaatacaaaactattcaaagagattgagtacgtggtggagtacccttggcacatgagtatcccacgcttagaagccagaagttatattgattcatatgacgacaattatgtatggcagaggaagactctatatagaatgccatctttgagtaattcaaaatgtttagaattggcaaaattggacttcaatatcgtacaatctttgcatcaagaggagttgaagcttctaacaagatggtggaaggaatccggcatggcagatataaatttcactcgacaccgagtggcggaggtttatttttcatcagctacatttgaacccgaatattctgccactagaattgccttcacaaaaattggttgtttacaagtcctttttgatgatatggctgacatctttgcaacactagatgaattgaaaagtttcactgagggagtaaagagatgggatacatctttgctacatgagattccagagtgtatgcaaacttgctttaaagtttggttcaaattaatggaagaagtaaataatgatgtggttaaggtacaaggacgtgacatgctcgctcacataagaaaaccctgggagttgtacttcaattgttatgtacaagaaagggagtggcttgaagccgggtatataccaacttttgaagagtacttaaagacttatgctatatcagtaggccttggaccgtgtaccctacaaccaatactactaatgggtgagcttgtgaaagatgatgttgttgagaaagtgcactatccctcaaatatgtttgagcttgtatccttgagctggcgactaacaaacgacaccaaaacatatcaggctgaaaaggctcgaggacaacaagcctcaggcatagcatgctatatgaaggataatccaggagcaactgaggaagatgccattaagcacatatgtcgtgttgttgatcgggccttgaaagaagcaagctttgaatatttcaaaccatccaatgatatcccaatgggttgcaagtcctttatttttaaccttagattgtgtgtccaaatcttttacaagtttatagatgggtacggaatcgccaatgaggagattaaggactatataagaaaagtttatattgatccaattcaagtatga

SEQ ID NO: 91 - DNA, 891 bp, synthetic construct
  misc_feature 1..891: note = Synthetic Polynucleotide
  source 1..891: mol_type = other DNA
atgtttgatttcaatgaatatatgaaaagtaaggctgttgcggtagacgcggctctggataaagcgattccgctggaatatcccgagaagattcacgaatcgatgcgctactccctgttagcaggagggaaacgcgttcgtccggcattatgcatcgcggcctgtgaactcgtcggcggttcacaggacttagcaatgccaactgcttgcgcaatggaaatgattcacacaatgagcctgattcatgatgatttgccttgcatggacaacgatgactttcggcgcggtaaacctactaatcataaggtttttggcgaagatactgcagtgctggcgggcgatgcgctgctgtcgtttgccttcgaacatatcgccgtcgcgacctcgaaaaccgtcccgtcggaccgtacgcttcgcgtgatttccgagctgggaaagaccatcggctctcaaggactcgtgggtggtcaggtagttgatatcacgtctgagggtgacgcgaacgtggacctgaaaaccctggagtggatccatattcacaaaacggccgtgctgctggaatgtagcgtggtgtcaggggggatcttggggggcgccacggaggatgaaatcgcgcgtattcgtcgttatgcccgctgtgttggactgttatttcaggtggtggatgacatcctggatgtcacaaaatccagcgaagagcttggcaagaccgcgggcaaagaccttctgacggataaggctacatacccgaaattgatgggcttggagaaagccaaggagttcgcagctgaacttgccacgcgggcgaaggaagaactctcttctttcgatcaaatcaaagccgcgccactgctgggcctcgccgattacattgcgtttcgtcagaactga

SEQ ID NO: 92 - DNA, 3150 bp, synthetic construct
  misc_feature 1..3150: note = Synthetic Polynucleotide
  source 1..3150: mol_type = other DNA
atgacaattaaagaaatgcctcagccaaaaacgtttggagagcttaaaaatttaccgttattaaacacagataaaccggttcaagctttgatgaaaattgcggatgaattaggagaaatctttaaattcgaggcgcctggtcgtgtaacgcgctacttatcaagtcagcgtctaattaaagaagcatgcgatgaatcacgctttgataaaaacttaagtcaagcgcttaaatttgtacgtgattttgcaggagacgggttatttacaagctggacgcatgaaaaaaattggaaaaaagcgcataatatcttacttccaagcttcagtcagcaggcaatgaaaggctatcatgcgatgatggtcgatatcgccgtgcagcttgttcaaaagtgggagcgtctaaatgcagatgagcatattgaagtaccggaagacatgacacgtttaacgcttgatacaattggtctttgcggctttaactatcgctttaacagcttttaccgagatcagcctcatccatttattacaagtatggtccgtgcactggatgaagcaatgaacaagctgcagcgagcaaatccagacgacccagcttatgatgaaaacaagcgccagtttcaagaagatatcaaggtgatgaacgacctagtagataaaattattgcagatcgcaaagcaagcggtgaacaaagcgatgatttattaacgcatatgctaaacggaaaagatccagaaacgggtgagccgcttgatgacgagaacattcgctatcaaattattacattcttaattgcgggacacgaaacaacaagtggtcttttatcatttgcgctgtatttcttagtgaaaaatccacatgtattacaaaaagcagcagaagaagcagcacgagttctagtagatcctgttccaagctacaaacaagtcaaacagcttaaatatgtcggcatggtcttaaacgaagcgctgcgcttatggccaactgctcctgcgttttccctatatgcaaaagaagatacggtgcttggaggagaatatcctttagaaaaaggcgacgaactaatggttctgattcctcagcttcaccgtgataaaacaatttggggagacgatgtggaagagttccgtccagagcgttttgaaaatccaagtgcgattccgcagcatgcgtttaaaccgtttggaaacggtcagcgtgcgtgtatcggtcagcagttcgctcttcatgaagcaacgctggtacttggtatgatgctaaaacactttgactttgaagatcatacaaactacgagctggatattaaagaaactttaacgttaaaacctgaaggctttgtggtaaaagcaaaatcgaaaaaaattccgcttggcggtattccttcacctagcactgaacagtctgctaaaaaagtacgcaaaaaggcagaaaacgctcataatacgccgctgcttgtgctatacggttcaaatatgggaacagctgaaggaacggcgcgtgatttagcagatattgcaatgagcaaaggatttgcaccgcaggtcgcaacgcttgattcacacgccggaaatcttccgcgcgaaggagctgtattaattgtaacggcgtcttataacggtcatccgcctgataacgcaaagcaatttgtcgactggttagaccaagcgtctgctgatgaagtaaaaggcgttcgctactccgtatttggatgcggcgataaaaactgggctactacgtatcaaaaagtgcctgcttttatcgatgaaacgcttgccgctaaaggggcagaaaacatcgctgaccgcggtgaagcagatgcaagcgacgactttgaaggcacatatgaagaatggcgtgaacatatgtggagtgacgtagcagcctactttaacctcgacattgaaaacagtgaagataataaatctactctttcacttcaatttgtcgacagcgccgcggatatgccgcttgcgaaaatgcacggtgcgttttcaacgaacgtcgtagcaagcaaagaacttcaacagccaggcagtgcacgaagcacgcgacatcttgaaattgaacttccaaaagaagcttcttatcaagaaggagatcatttaggtgttattcctcgcaactatgaaggaatagtaaaccgtgtaacagcaaggttcggcctagatgcatcacagcaaatccgtctggaagcagaagaagaaaaattagctcatttgccactcgctaaaacagtatccgtagaagagcttctgcaatacgtggagcttcaagatcctgttacgcgcacgcagcttcgcgcaatggctgctaaaacggtctgcccgccgcataaagtagagcttgaagccttgcttgaaaagcaagcctacaaagaacaagtgctggcaaaacgtttaacaatgcttgaactgcttgaaaaatacccggcgtgtgaaatgaaattcagcgaatttatcgcccttctgccaagcatacgcccgcgctattactcgatttcttcatcacctcgtgtcgatgaaaaacaagcaagcatcacggtcagcgttgtctcaggagaagcgtggagcggatatggagaatataaaggaattgcgtcgaactatcttgccgagctgcaagaaggagatacgattacgtgctttatttccacaccgcagtcagaatttacgctgccaaaagaccctgaaacgccgcttatcatggtcggaccgggaacaggcgtcgcgccgtttagaggctttgtgcaggcgcgcaaacagctaaaagaacaaggacagtcacttggagaagcacatttatacttcggctgccgttcacctcatgaagactatctgtatcaagaagagcttgaaaacgcccaaagcgaaggcatcattacgcttcataccgctttttctcgcatgccaaatcagccgaaaacatacgttcagcacgtaatggaacaagacggcaagaaattgattgaacttcttgatcaaggagcgcacttctatatttgcggagacggaagccaaatggcacctgccgttgaagcaacgcttatgaaaagctatgctgacgttcaccaagtgagtgaagcagacgctcgcttatggctgcagcagctagaagaaaaaggccgatacgcaaaagacgtgtgggctgggtaa

SEQ ID NO: 93 - DNA, 789 bp, synthetic construct
  misc_feature 1..789: note = Synthetic Polynucleotide
  source 1..789: mol_type = other DNA
atgagggaagcggtgatcgccgaagtatcgactcaactatcagaggtagttggcgtcatcgagcgccatctcgaaccgacgttgctggccgtacatttgtacggctccgcagtggatggcggcctgaagccacacagtgatattgatttgctggttacggtgaccgtaaggcttgatgaaacaacgcggcgagctttgatcaacgaccttttggaaacttcggcttcccctggagagagcgagattctccgcgctgtagaagtcaccattgttgtgcacgacgacatcattccgtggcgttatccagctaagcgcgaactgcaatttggagaatggcagcgcaatgacattcttgcaggtatcttcgagccagccacgatcgacattgatctggctatcttgctgacaaaagcaagagaacatagcgttgccttggtaggtccagcggcggaggaactctttgatccggttcctgaacaggatctatttgaggcgctaaatgaaaccttaacgctatggaactcgccgcccgactgggctggcgatgagcgaaatgtagtgcttacgttgtcccgcatttggtacagcgcagtaaccggcaaaatcgcgccgaaggatgtcgctgccgactgggcaatggagcgcctgccggcccagtatcagcccgtcatacttgaagctagacaggcttatcttggacaagaagaagatcgcttggcctcgcgcgcagatcagttggaagaatttgtccactacgtgaaaggcgagatcaccaaggtagtcggcaaa

SEQ ID NO: 94 - DNA, 432 bp, synthetic construct
  misc_feature 1..432: note = Synthetic Polynucleotide
  source 1..432: mol_type = other DNA
ttggctactacacttgaacgtattgagaagaactttgtcattactgacccaaggttgccagataatcccattatattcgcgtccgatagtttcttgcagttgacagaatatagccgtgaagaaattttgggaagaaactgcaggtttctacaaggtcctgaaactgatcgcgcgacagtgagaaaaattagagatgccatagataaccaaacagaggtcactgttcagctgattaattatacaaagagtggtaaaaagttctggaacctctttcacttgcagcctatgcgagatcagaagggagatgtccagtactttattggggttcagttggatggaactgagcatgtccgagatgctgccgagagagagggagtcatgctgattaagaaaactgcagaaaatattgatgaggcggcaaaagaacttcca

SEQ ID NO: 95 - DNA, 2244 bp, synthetic construct
  misc_feature 1..2244: note = Synthetic Polynucleotide
  source 1..2244: mol_type = other DNA
atggctagcgtggcaggtcatgcctctggcagccccgcattcgggaccgccgatctttcgaattgcgaacgtgaagagatccacctcgccggctcgatccagccgcatggcgcgcttctggtcgtcagcgagccggatcatcgcatcatccaggccagcgccaacgccgcggaatttctgaatctcggaagcgtgctcggcgttccgctcgccgagatcgacggcgatctgttgatcaagatcctgccgcatctcgatcccaccgccgaaggcatgccggtcgcggtgcgctgccggatcggcaatccctccacggagtacgacggtctgatgcatcggcctccggaaggcgggctgatcatcgagctcgaacgtgccggcccgccgatcgatctgtccggcacgctggcgccggcgctggagcggatccgcacggcgggctcgctgcgcgcgctgtgcgatgacaccgcgctgctgtttcagcagtgcaccggctacgaccgggtgatggtgtatcgcttcgacgagcagggccacggcgaagtgttctccgagcgccacgtgcccgggctcgaatcctatttcggcaaccgctatccgtcgtcggacattccgcagatggcgcggcggctgtacgagcggcagcgcgtccgcgtgctggtcgacgtcagctatcagccggtgccgctggagccgcggctgtcgccgctgaccgggcgcgatctcgacatgtcgggctgcttcctgcgctcgatgtcgccgatccatctgcagtacctgaagaacatgggcgtgcgcgccaccctggtggtgtcgctggtggtcggcggcaagctgtggggcctggttgcctgtcatcattatctgccgcgcttcatgcatttcgagctgcgggcgatctgcgaactgctcgccgaagcgatcgcgacgcggatcaccgcgcttgagagcttcgcgcagagccagtcggagctgttcgtgcagcggctcgaacagcgcatgatcgaagcgattacccgtgaaggcgattggcgcgcagcgattttcgacaccagccaatcgatcctgcagccgctgcacgccgccggttgcgcgctggtgtacgaagaccagatcaggaccatcggcgacgtgccttccacgcaggatgtgcgcgagatcgccgggtggctcgatcgccagccgcgcgcggcggtgacctcgaccgcgtcgctcggtctcgacgtgccggagctcgcgcatctgacgcggatggcgagcggcgtggtcgcggcgccgatttcggatcatcgcggcgagtttctgatgtggttccgccccgagcgcgtccacaccgttacctggggcggcgatccgaagaagccgttcacgatgggcgatacaccggcggatctgtcgccgcggcgctccttcgccaaatggcatcaggttgtcgaaggcacgtccgatccgtggacggccgccgatctcgccgcggctcgcaccatcggtcagaccgtcgccgacatcgtgctgcaattccgcgcggtgcggacactgatcgcccgcgaacagtacgaacagttttcgtcccaggtgcacgcttcgatgcagccggtgctgatcaccgacgccgaaggccgcatcctgctgatgaacgactcgttccgcgacatgttgccggcgggttcgccatccgccgtccatctcgacgatctcgccgggttcttcgtcgaatcgaacgatttcctgcgcaacgtcgccgaactgatcgatcacggccgcgggtggcgcggcgaagttctgctgcgcggcgcaggcaaccgcccgttgccgctggcagtgcgcgccgatccggtgacgcgcacggaggaccagtcgctcggcttcgtgctgatcttcagcgacgctaccgatcgtcgcaccgcagatgccgcacgcacgcgtttccaggaaggcattcttgccagcgcacgtcccggcgtgcggctcgactccaagtccgacctgttgcacgagaagctgctgtccgcgctggtcgagaacgcgcagcttgccgcattggaaatcacttacggcgtcgagaccggacgcatcgccgagctgctcgaaggcgtccgccagtcgatgctgcgcaccgccgaagtgctcggccatctggtgcagcacgcggcgcgcacggccggcagcgacagctcgagcaatggctcgcagaacaagaaggaattcgatagtgctggtagtgctggtagtgctggtactagt

SEQ ID NO: 96 - DNA, 1308 bp, synthetic construct; identical to SEQ ID NO: 75
  misc_feature 1..1308: note = Synthetic Polynucleotide
  source 1..1308: mol_type = other DNA

SEQ ID NO: 97 - DNA, 951 bp, synthetic construct
  misc_feature 1..951: note = Synthetic Polynucleotide
  source 1..951: mol_type = other DNA
atgcccaccaccatcgagcgggagttcgaagagttggatactcagcgtcgctggcagccgctgtacttggaaattcgaaatgagtcccatgactatcctcatagagtggccaagtttccagaaaacagaaatcgaaacagatacagagatgtaagcccatatgatcacagtcgtgttaaactgcaaaatgctgagaatgattatattaatgccagtttagttgacatagaagaggcacaaaggagttacatcttaacacagggtccacttcctaacacatgctgccatttctggcttatggtttggcagcagaagaccaaagcagttgtcatgctgaaccgcattgtggagaaagaatcggttaaatgtgcacagtactggccaacagatgaccaagagatgctgtttaaagaaacaggattcagtgtgaagctcttgtcagaagatgtgaagtcgtattatacagtacatctactacaattagaaaatatcaatagtggtgaaaccagaacaatatctcactttcattatactacctggccagattttggagtccctgaatcaccagcttcatttctcaatttcttgtttaaagtgagagaatctggctccttgaaccctgaccatgggcctgcggtgatccactgtagtgcaggcattgggcgctctggcaccttctctctggtagacacttgtcttgttttgatggaaaaaggagatgatattaacataaaacaagtgttactgaacatgagaaaataccgaatgggtcttattcagaccccagatcaactgagattctcatacatggctataatagaaggagcaaaatgtataaagggagattctagtatacagaaacgatggaaagaactttctaaggaagacttatctcctgcctttgatcattcaccaaacaaaataatgactgaaaaatacaatgggaacaga

SEQ ID NO: 98 - DNA, 900 bp, synthetic construct
  misc_feature 1..900: note = Synthetic Polynucleotide
  source 1..900: mol_type = other DNA
atgtcttctggtgtagatctgggtaccgagaacctgtacttccaatccatgtcccgtgtcctccaagcagaagagcttcatgaaaaggccctggaccctttcctgctgcaggcggaattctttgaaatccccatgaactttgtggatccgaaagagtacgacatccctgggctggtgcggaagaaccggtacaaaaccatacttcccaaccctcacagcagagtgtgtctgacctcaccagaccctgacgaccctctgagttcctacatcaatgccaactacatccggggctatggtggggaggagaaggtgtacatcgccactcagggacccatcgtcagcacggtcgccgacttctggcgcatggtgtggcaggagcacacgcccatcattgtcatgatcaccaacatcgaggagatgaacgagaaatgcaccgagtattggccggaggagcaggtggcgtacgacggtgttgagatcactgtgcagaaagtcattcacacggaggattaccggctgcgactcatctccctcaagagtgggactgaggagcgaggcctgaagcattactggttcacatcctggcccgaccagaagaccccagaccgggcccccccactcctgcacctggtgcgggaggtggaggaggcagcccagcaggaggggccccactgtgcccccatcatcgtccactgcagtgcagggattgggaggaccggctgcttcattgccaccagcatctgctgccagcagctgcggcaggagggtgtagtggacatcctgaagaccacgtgccagctccgtcaggacaggggcggcatgatccagacatgcgagcagtaccagtttgtgcaccacgtcatgagcctctacgaaaagcagctgtcccaccagtcctga

SEQ ID NO: 99 - DNA, 1788 bp, synthetic construct
  misc_feature 1..1788: note = Synthetic Polynucleotide
  source 1..1788: mol_type = other DNA
atggtgaggtggtttcaccgagacctcagtgggctggatgcagagaccctgctcaagggccgaggtgtccacggtagcttcctggctcggcccagtcgcaagaaccagggtgacttctcgctctccgtcagggtgggggatcaggtgacccatattcggatccagaactcaggggatttctatgacctgtatggaggggagaagtttgcgactctgacagagctggtggagtactacactcagcagcagggtgtggtgcaggaccgcgacggcaccatcatccacctcaagtacccgctgaactgctccgatcccactagtgagaggtggtaccatggccacatgtctggcgggcaggcagagacgctgctgcaggccaagggcgagccctggacgtttcttgtgcgtgagagcctcagccagcctggagacttcgtgctttctgtgctcagtgaccagcccaaggctggcccaggctccccgctcagggtcacccacatcaaggtcatgtgcgagggtggacgctacacagtgggtggtttggagaccttcgacagcctcacggacctggtggagcatttcaagaagacggggattgaggaggcctcaggcgcctttgtctacctgcggcagccgtactatgccacgagggtgaatgcggctgacattgagaaccgagtgttggaactgaacaagaagcaggagtccgaggatacagccaaggctggcttctgggaggagtttgagagtttgcagaagcaggaggtgaagaacttgcaccagcgtctggaagggcaacggccagagaacaagggcaagaaccgctacaagaacattctcccctttgaccacagccgagtgatcctgcagggacgggacagtaacatccccgggtccgactacatcaatgccaactacatcaagaaccagctgctaggccctgatgagaacgctaagacctacatcgccagccagggctgtctggaggccacggtcaatgacttctggcagatggcgtggcaggagaacagccgtgtcatcgtcatgaccacccgagaggtggagaaaggccggaacaaatgcgtcccatactggcccgaggtgggcatgcagcgtgcttatgggccctactctgtgaccaactgcggggagcatgacacaaccgaatacaaactccgtaccttacaggtctccccgctggacaatggagacctgattcgggagatctggcattaccagtacctgagctggcccgaccatggggtccccagtgagcctgggggtgtcctcagcttcctggaccagatcaaccagcggcaggaaagtctgcctcacgcagggcccatcatcgtgcactgcagcgccggcatcggccgcacaggcaccatcattgtcatcgacatgctcatggagaacatctccaccaagggcctggactgtgacattgacatccagaagaccatccagatggtgcgggcgcagcgctcgggcatggtgcagacggaggcgcagtacaagttcatctacgtggccatcgcccagttcattgaaaccactaagaagaagctggaggtcctgcagtcgcagaagggccaggagtcggagtacgggaacatcacctatcccccagccatgaagaatgcccatgccaaggcctcccgcacctcgtccaaacacaaggaggatgtgtatgagaacctgcacactaagaacaagagggaggagaaagtgaagaagcagcggtcagcagacaaggagaagagcaagggttccctcaagaggaagtga

SEQ ID NO: 100 - DNA, 1782 bp, synthetic construct
  misc_feature 1..1782: note = Synthetic Polynucleotide
  source 1..1782: mol_type = other DNA
atgacatcgcggagatggtttcacccaaatatcactggtgtggaggcagaaaacctactgttgacaagaggagttgatggcagttttttggcaaggcctagtaaaagtaaccctggagacttcacactttccgttagaagaaatggagctgtcacccacatcaagattcagaacactggtgattactatgacctgtatggaggggagaaatttgccactttggctgagttggtccagtattacatggaacatcacgggcaattaaaagagaagaatggagatgtcattgagcttaaatatcctctgaactgtgcagatcctacctctgaaaggtggtttcatggacatctctctgggaaagaagcagagaaattattaactgaaaaaggaaaacatggtagttttcttgtacgagagagccagagccaccctggagattttgttctttctgtgcgcactggtgatgacaaaggggagagcaatgacggcaagtctaaagtgacccatgttatgattcgctgtcaggaactgaaatacgacgttggtggaggagaacggtttgattctttgacagatcttgtggaacattataagaagaatcctatggtggaaacattgggtacagtactacaactcaagcagccccttaacacgactcgtataaatgctgctgaaatagaaagcagagttcgagaactaagcaaattagctgagaccacagataaagtcaaacaaggcttttgggaagaatttgagacactacaacaacaggagtgcaaacttctctacagccgaaaagagggtcaaaggcaagaaaacaaaaacaaaaatagatataaaaacatcctgccctttgatcataccagggttgtcctacacgatggtgatcccaatgagcctgtttcagattacatcaatgcaaatatcatcatgcctgaatttgaaaccaagtgcaacaattcaaagcccaaaaagagttacattgccacacaaggctgcctgcaaaacacggtgaatgacttttggcggatggtgttccaagaaaactcccgagtgattgtcatgacaacgaaagaagtggagagaggaaagagtaaatgtgtcaaatactggcctgatgagtatgctctaaaagaatatggcgtcatgcgtgttaggaacgtcaaagaaagcgccgctcatgactatacgctaagagaacttaaactttcaaaggttggacaagggaatacggagagaacggtctggcaataccactttcggacctggccggaccacggcgtgcccagcgaccctgggggcgtgctggacttcctggaggaggtgcaccataagcaggagagcatcatggatgcagggccggtcgtggtgcactgcagtgctggaattggccggacagggacgttcattgtgattgatattcttattgacatcatcagagagaaaggtgttgactgcgatattgacgttcccaaaaccatccagatggtgcggtctcagaggtcagggatggtccagacagaagcacagtaccgatttatctatatggcggtccagcattatattgaaacactacagcgcaggattgaagaagagcagaaaagcaagaggaaagggcacgaatatacaaatattaagtattctctagcggaccagacgagtggagatcagagccctctcccgccttgtactccaacgccaccctgtgcagaaatgagagaagacagtgctagagtctatgaaaacgtgggcctgatgcaacagcagaaaagtttcagatga

SEQ ID NO: 101 - DNA, 1275 bp, synthetic construct
  misc_feature 1..1275: note = Synthetic Polynucleotide
  source 1..1275: mol_type = other DNA
atggagcaagtggagatcctgaggaaattcatccagagggtccaggccatgaagagtcctgaccacaatggggaggacaacttcgcccgggacttcatgcggttaagaagattgtctaccaaatatagaacagaaaagatatatcccacagccactggagaaaaagaagaaaatgttaaaaagaacagatacaaggacatactgccatttgatcacagccgagttaaattgacattaaagactccttcacaagattcagactatatcaatgcaaattttataaagggcgtctatgggccaaaagcatatgtagcaactcaaggacctttagcaaatacagtaatagatttttggaggatggtatgggagtataatgttgtgatcattgtaatggcctgccgagaatttgagatgggaaggaaaaaatgtgagcgctattggcctttgtatggagaagaccccataacgtttgcaccatttaaaatttcttgtgaggatgaacaagcaagaacagactacttcatcaggacactcttacttgaatttcaaaatgaatctcgtaggctgtatcagtttcattatgtgaactggccagaccatgatgttccttcatcatttgattctattctggacatgataagcttaatgaggaaatatcaagaacatgaagatgttcctatttgtattcattgcagtgcaggctgtggaagaacaggtgccatttgtgccatagattatacgtggaatttactaaaagctgggaaaataccagaggaatttaatgtatttaatttaatacaagaaatgagaacacaaaggcattctgcagtacaaacaaaggagcaatatgaacttgttcatagagctattgcccaactgtttgaaaaacagctacaactatatgaaattcatggagctcagaaaattgctgatggagtgaatgaaattaacactgaaaacatggtcagctccatagagcctgaaaaacaagattctcctcctccaaaaccaccaaggacccgcagttgccttgttgaaggggatgctaaagaagaaatactgcagccaccggaacctcatccagtgccacccatcttgacaccttctcccccttcagcttttccaacagtcactactgtgtggcaggacaatgatagataccatccaaagccagtgttgcaatggtttcatcagaacaacattcagcagacctcaacagaaactatagtaaatcaacagaacttccagggaaaaatgaatcaacaattgaacaga

SEQ ID NO: 102 - DNA, 899 bp, synthetic construct
  misc_feature 1..899: note = Synthetic Polynucleotide
  source 1..899: mol_type = other DNA
atggaccaaagagaaattctgcagaagttcctggatgaggcccaaagcaagaaaattactaaagaggagtttgccaatgaatttctgaagctgaaaaggcaatctaccaagtacaaggcagacaaaacctatcctacaactgtggctgagaagcccaagaatatcaagaaaaacagatataaggatattttgccctatgattatagccgggtagaactatccctgataacctctgatgaggattccagctacatcaatgccaacttcattaagggagtttatggacccaaggcttatattgccacccagggtcctttatctacaaccctcctggacttctggaggatgatttgggaatatagtgtccttatcattgttatggcatgcatggagtatgaaatgggaaagaaaaagtgtgagcgctactgggctgagccaggagagatgcagctggaatttggccctttctctgtatcctgtgaagctgaaaaaaggaaatctgattatataatcaggactctaaaagttaagttcaatagtgaaactcgaactatctaccagtttcattacaagaattggccagaccatgatgtaccttcatctatagaccctattcttgagctcatctgggatgtacgttgttaccaagaggatgacagtgttcccatatgcattcactgcagtgctggctgtggaaggactggtgttatttgtgctattgattatacatggatgttgctaaaagatgggataattcctgagaacttcagtgttttcagtttgatccgggaaatgcggacacagaggccttcattagttcaaacgcaggaacaatatgaactggtctacaatgctgtattagaactatttaagagacagatggatgttatcagagataa

SEQ ID NO: 103 - DNA, 1149 bp, synthetic construct
  misc_feature 1..1149: note = Synthetic Polynucleotide
  source 1..1149: mol_type = other DNA
atgagtctgaaagaaaaaacacaatctctgtttgccaacgcatttggctaccctgccactcacaccattcaggcgcctggccgcgtgaatttgattggtgaacacaccgactacaacgacggtttcgttctgccctgcgcgattgattatcaaaccgtgatcagttgtgcaccacgcgatgaccgtaaagttcgcgtgatggcagccgattatgaaaatcagctcgacgagttttccctcgatgcgcccattgtcgcacatgaaaactatcaatgggctaactacgttcgtggcgtggtgaaacatctgcaactgcgtaacaacagcttcggcggcgtggacatggtgatcagcggcaatgtgccgcagggtgccgggttaagttcttccgcttcactggaagtcgcggtcggaaccgtattgcagcagctttatcatctgccgctggacggcgcacaaatcgcgcttaacggtcaggaagcagaaaaccagtttgtaggctgtaactgcgggatcatggatcagctaatttccgcgctcggcaagaaagatcatgccttgctgatcgattgccgctcactggggaccaaagcagtttccatgcccaaaggtgtggctgtcgtcatcatcaacagtaacttcaaacgtaccctggttggcagcgaatacaacacccgtcgtgaacagtgcgaaaccggtgcgcgtttcttccagcagccagccctgcgtgatgtcaccattgaagagttcaacgctgttgcgcatgaactggacccgatcgtggcaaaacgcgtgcgtcatatactgactgaaaacgcccgcaccgttgaagctgccagcgcgctggagcaaggcgacctgaaacgtatgggcgagttgatggcggagtctcatgcctctatgcgcgatgatttcgaaatcaccgtgccgcaaattgacactctggtagaaatcgtcaaagctgtgattggcgacaaaggtggcgtacgcatgaccggcggcggatttggcggctgtatcgtcgcgctgatcccggaagagctggtgcctgccgtacagcaagctgtcgctgaacaatatgaagcaaaaacaggtattaaagagactttttacgtttgtaaaccatcacaaggagcaggacagtgctga

SEQ ID NO: 104 - DNA, 1422 bp, synthetic construct
  misc_feature 1..1422: note = Synthetic Polynucleotide
  source 1..1422: mol_type = other DNA
atgaacatcaaaaagtttgcaaaacaagcaacagtattaacctttactaccgcactgctggcaggaggcgcaactcaagcgtttgcgaaagaaacgaaccaaaagccatataaggaaacatacggcatttcccatattacacgccatgatatgctgcaaatccctgaacagcaaaaaaatgaaaaatatcaagttcctgaattcgattcgtccacaattaaaaatatctcttctgcaaaaggcctggacgtttgggacagctggccattacaaaacgctgacggcactgtcgcaaactatcacggctaccacatcgtctttgcattagccggagatcctaaaaatgcggatgacacatcgatttacatgttctatcaaaaagtcggcgaaacttctattgacagctggaaaaacgctggccgcgtctttaaagacagcgacaaattcgatgcaaatgattctatcctaaaagaccaaacacaagaatggtcaggttcagccacatttacatctgacggaaaaatccgtttattctacactgatttctccggtaaacattacggcaaacaaacactgacaactgcacaagttaacgtatcagcatcagacagctctttgaacatcaacggtgtagaggattataaatcaatctttgacggtgacggaaaaacgtatcaaaatgtacagcagttcatcgatgaaggcaactacagctcaggcgacaaccatacgctgagagatcctcactacgtagaagataaaggccacaaatacttagtatttgaagcaaacactggaactgaagatggctaccaaggcgaagaatctttatttaacaaagcatactatggcaaaagcacatcattcttccgtcaagaaagtcaaaaacttctgcaaagcgataaaaaacgcacggctgagttagcaaacggcgctctcggtatgattgagctaaacgatgattacacactgaaaaaagtgatgaaaccgctgattgcatctaacacagtaacagatgaaattgaacgcgcgaacgtctttaaaatgaacggcaaatggtacctgttcactgactcccgcggatcaaaaatgacgattgacggcattacgtctaacgatatttacatgcttggttatgtttctaattctttaactggcccatacaagccgctgaacaaaactggccttgtgttaaaaatggatcttgatcctaacgatgtaacctttacttactcacacttcgctgtacctcaagcgaaaggaaacaatgtcgtgattacaagctatatgacaaacagaggattctacgcagacaaacaatcaacgtttgcgccaagcttcctgctgaacatcaaaggcaagaaaacatctgttgtcaaagacagcatccttgaacaaggacaattaacagttaacaaataa